European Patent Application EP 4 775 679 A2, published July 15, 2026. Title: CpG REDUCED FACTOR VIII VARIANTS, COMPOSITIONS AND METHODS AND USES FOR TREATMENT OF HEMOSTASIS DISORDERS. Applicant: SPARK THERAPEUTICS, INC. Application EP. The sequence listing filed with the application follows.

SEQUENCE LISTING (29 sequences)

SEQ ID NO: 1 - DNA, 4374 bp, synthetic construct
  misc_feature 1..4374: note = Description of Artificial Sequence: FVIII Nucleic Acid
  source 1..4374: mol_type = other DNA
atgcagattgagctgtctacctgcttcttcctgtgcctgctgaggttctgcttctctgctaccaggaggtactacctgggggctgtggagctgagctgggattacatgcagtctgacctgggggagctgcctgtggatgccaggtttccccccagggtgcccaagagcttccccttcaatacctctgtggtgtataagaagaccctgtttgtggagttcactgatcatctgttcaacattgctaaacccaggcccccctggatggggctgctgggccctaccatccaggctgaggtgtatgacactgtggtgatcactctgaagaacatggctagccatcctgtgtctctgcatgctgtgggggtgagctactggaaggcttctgagggggctgagtatgatgatcagactagccagagggagaaggaggatgacaaggtgttccctgggggctctcacacctatgtctggcaggtgctgaaggagaatggccccatggcctctgatcctctgtgtctgacctatagctacctgagccatgtggacctggtgaaggacctgaactctggcctgattggggccctgctggtgtgtagggaggggagcctggccaaggagaagacccagaccctgcacaagttcattctgctgtttgctgtgtttgatgagggcaagagctggcattctgaaaccaagaacagcctgatgcaggacagggatgctgcctctgctagggcctggcccaagatgcacactgtgaatgggtatgtcaataggtctctgcctggcctgattggctgccacaggaagtctgtgtactggcatgtgattgggatgggcaccacccctgaggtgcacagcatctttctggagggccacaccttcctggtgaggaatcacagacaggccagcctggagatcagccccatcaccttcctgactgcccagaccctgctgatggacctgggccagtttctgctgttctgccacatctctagccaccagcatgatggcatggaggcctatgtgaaggtggactcctgccctgaggagccccagctgaggatgaagaataatgaggaggctgaggactatgatgatgacctgactgactctgagatggatgtggtgagatttgatgatgacaattctcccagcttcattcagatcaggtctgtggccaagaagcatcccaagacctgggtgcactacattgctgctgaggaggaggactgggactatgcccccctggtgctggcccctgatgacaggagctataagagccagtacctgaataatggcccccagaggattgggaggaagtataagaaggtgaggttcatggcctatactgatgaaaccttcaagaccagagaggccatccagcatgagtctgggatcctggggcccctgctgtatggggaggtgggggacaccctgctgatcatcttcaagaaccaggccagcaggccctacaacatctaccctcatggcatcactgatgtgaggcctctgtacagcagaaggctgcccaagggggtgaagcatctgaaggacttccccattctgcctggggagattttcaagtacaagtggactgtgactgtggaggatggcccaaccaagtctgaccctaggtgcctgactaggtactacagcagctttgtgaatatggagagggacctggcctctggcctgattggccccctgctgatctgctacaaggagtctgtggatcagaggggcaaccagatcatgtctgacaagaggaatgtgatcctgttctctgtgtttgatgagaacaggagctggtacctgactgagaacattcagaggtttctgcccaaccctgctggggtgcagctggaggaccctgaattccaggcctctaacatcatgcacagcattaatggctatgtgtttgacagcctgcagctgtctgtgtgcctgcatgaggtggcctactggtacattctgagcattggggcccagactgacttcctgtctgtgttcttctctggctacacctttaagcacaagatggtgtatgaggataccctgaccctgtttcctttctctggggagactgtgttcatgagcatggagaaccctggcctgtggatcctgggctgccacaactctgacttcaggaacagggggatgactgctctgctgaaggtgagcagctgtgataagaacactggggactactatgaggacagctatgaggacatctctgcctatctgctgagcaagaataatgctattgagcccaggagcttctctcagaacccccctgtgctgaagaggcaccagagggagatcaccagaactactctgcagtctgaccaggaggagattgactatgatgacaccatctctgtggagatgaagaaggaggattttgatatttatgatgaggatgaaaaccagagccccaggagctttcagaagaagactaggcactatttcattgctgctgtggagaggctgtgggactatggcatgtcttctagcccccatgtgctgaggaacagggcccagtctggctctgtgccccagttcaagaaggtggtgttccaggagttcactgatggcagcttcactcagcccctgtacaggggggagctgaatgagcacctggggctgctgggcccttatatcagggctgaggtggaggataacatcatggtgaccttcaggaaccaggccagcaggccctacagcttctactctagcctgatcagctatgaggaggaccagaggcagggggctgagcccaggaagaactttgtgaagcccaatgagaccaagacttatttctggaaggtgcagcaccatatggcccccaccaaggatgagtttgattgcaaagcctgggcctacttctctgatgtggacctggagaaggatgtgcactctgggctgattggccccctgctggtgtgccacaccaacactctgaaccctgcccatggcaggcaggtgactgtgcaggagtttgccctgttcttcaccatctttgatgagactaagagctggtacttcactgagaacatggagaggaactgcagggccccctgcaatatccagatggaggaccccacctttaaggaaaattataggtttcatgccattaatggctacatcatggacaccctgcctggcctggtgatggcccaggaccagaggatcaggtggtacctgctgagcatgggcagcaatgagaacattcacagcatccacttctctggccatgtgttcactgtgaggaagaaggaggagtacaagatggccctgtataatctgtaccctggggtgtttgagactgtggagatgctgcccagcaaggctggcatctggagggtggagtgcctgattggggagcacctgcatgctggcatgagcaccctgttcctggtgtattctaacaagtgtcagacccccctgggcatggcctctggccatatcagggacttccagatcactgcctctggccagtatgggcagtgggcccccaagctggccaggctgcattactctggcagcatcaatgcctggagcaccaaggagccattcagctggattaaggtggacctgctggctccaatgattatccatggcatcaagacccagggggccaggcagaagtttagcagcctgtacatctctcagtttatcatcatgtactctctggatggcaaaaagtggcagacctacaggggcaattctactggcactctgatggtgttctttggcaatgtggacagctctgggatcaagcacaacatctttaacccccctatcattgccaggtacattaggctgcaccccacccattacagcatcaggagcaccctgaggatggagctgatgggctgtgatctgaacagctgcagcatgcccctgggcatggagagcaaggctatctctgatgcccagattactgccagcagctacttcaccaatatgtttgccacctggagccccagcaaggccaggctgcacctgcagggcaggtctaatgcctggaggccccaggtgaacaaccccaaggagtggctgcaggtggacttccagaagaccatgaaggtgactggggtgaccacccagggggtgaagagcctgctgactagcatgtatgtgaaggagttcctgatcagcagcagccaggatggccatcagtggaccctgttcttccagaatggcaaggtgaaggtgttccagggcaatcaggacagcttcacccctgtggtgaacagcctggacccccccctgctgaccagatacctgaggatccacccccagagctgggtgcatcagattgccctgaggatggaggtgctggggtgtgaggcccaggacctgtactga

SEQ ID NO: 2 - DNA, 4374 bp, synthetic construct
  misc_feature 1..4374: note = Description of Artificial Sequence: FVIII Nucleic Acid
  source 1..4374: mol_type = other DNA
atgcagattgagctgtctacctgctttttcctgtgtctgctgaggttctgcttctctgccactaggaggtactacctgggggctgtggagctgtcttgggattacatgcagtctgatctgggggagctgcctgtggatgccaggtttcctcccagggtgcccaagtctttccccttcaatacctctgtggtgtataagaagaccctgtttgtggagtttactgatcacctgttcaacattgccaagcccaggcccccttggatgggcctgctggggcccaccatccaggctgaggtgtatgacactgtggtgatcaccctgaagaacatggcctctcaccctgtgagcctgcatgctgtgggggtgagctactggaaggcctctgagggggctgagtatgatgaccagaccagccagagggagaaggaggatgataaggtgttccctggggggagccacacttatgtgtggcaggtgctgaaggagaatggcccaatggcctctgatcccctgtgcctgacctattcttacctgagccatgtggacctggtgaaggacctgaactctggcctgattggggccctgctggtgtgcagggagggctctctggctaaggagaagacccagaccctgcacaagttcatcctgctgtttgctgtgtttgatgaggggaagagctggcactctgagaccaagaacagcctgatgcaggacagggatgctgcctctgccagggcctggcccaaaatgcacactgtgaatggctatgtgaataggagcctgcctggcctgattggctgccacaggaagtctgtgtattggcatgtgattggcatgggcaccacccctgaggtgcactctatcttcctggagggccatactttcctggtgaggaatcataggcaggccagcctggagattagccccattacctttctgactgcccagaccctgctgatggacctgggccagttcctgctgttttgccacatcagctctcaccagcatgatggcatggaggcctatgtgaaggtggatagctgccctgaggagccccagctgaggatgaagaacaatgaggaggctgaggattatgatgatgatctgactgattctgaaatggatgtggtgaggtttgatgatgacaatagcccctctttcatccagatcaggtctgtggccaagaagcatcctaagacctgggtgcactacattgctgctgaggaggaggactgggactatgctcccctggtgctggcccctgatgacaggtcttacaagagccagtacctgaacaatggcccccagagaattgggaggaagtataagaaggtgagattcatggcttacactgatgagaccttcaagactagggaggccatccagcatgagtctggcattctgggccccctgctgtatggggaggtgggggacaccctgctgatcatcttcaagaaccaggcctctaggccctacaatatttacccccatgggatcactgatgtgaggcccctgtacagcaggaggctgcctaagggggtgaagcatctgaaggacttccccatcctgcctggggagatcttcaagtataagtggactgtgactgtggaagatggccccaccaagtctgaccctaggtgcctgaccaggtactactcttcttttgtgaacatggagagggacctggcctctggcctgattggccccctgctgatctgctacaaggagtctgtggaccagagggggaaccagattatgtctgacaagaggaatgtgattctgttctctgtgtttgatgagaacaggagctggtatctgactgagaacatccagaggttcctgcccaatcctgctggggtgcagctggaggaccctgagttccaggccagcaacatcatgcacagcatcaatgggtatgtgtttgattctctgcagctgtctgtgtgcctgcatgaggtggcctactggtacatcctgagcattggggctcagactgatttcctgtctgtgttcttttctggctacacctttaagcataagatggtgtatgaggacactctgaccctgtttcccttctctggggagactgtgtttatgagcatggagaaccctggcctgtggatcctgggctgccacaactctgatttcaggaacaggggcatgactgctctgctgaaggtgtcttcttgtgacaagaacactggggactattatgaggacagctatgaggacatctctgcctacctgctgagcaagaacaatgctattgagcccagatctttcagccagaacccccctgtgctgaagaggcaccagagggagatcactaggaccaccctgcagtctgaccaggaggagattgactatgatgacactatctctgtggagatgaagaaggaggactttgatatctatgatgaggatgagaaccagtctcccaggagcttccagaaaaagaccaggcactacttcattgctgctgtggagaggctgtgggactatggcatgtcttctagcccccatgtgctgaggaacagggcccagtctgggtctgtgccccagttcaagaaggtggtgttccaggagttcactgatgggagcttcacccagcctctgtacaggggggagctgaatgagcacctggggctgctgggcccttatattagggctgaggtggaggacaacatcatggtgactttcaggaatcaggcctctaggccctatagcttctacagctctctgatcagctatgaggaggatcagaggcagggggctgagcccaggaagaactttgtgaagcccaatgagaccaagacctacttctggaaggtgcagcaccacatggctcctaccaaggatgagtttgactgcaaggcctgggcctacttttctgatgtggacctggagaaggatgtgcactctggcctgattggccccctgctggtgtgtcataccaacaccctgaaccctgcccatggcaggcaggtgactgtgcaggagtttgccctgttcttcaccatctttgatgagaccaagagctggtactttactgagaacatggagaggaattgcagagccccttgcaacatccagatggaggacccaaccttcaaagagaactacaggttccatgccatcaatgggtacatcatggacaccctgcctggcctggtgatggctcaggaccagaggatcaggtggtatctgctgagcatgggcagcaatgagaatatccatagcattcacttctctggccatgtgttcactgtgaggaagaaggaggagtacaagatggccctgtataacctgtaccctggggtgtttgagactgtggagatgctgccaagcaaggctgggatttggagggtggagtgcctgattggggagcacctgcatgctggcatgtctaccctgttcctggtgtactccaataagtgccagacccccctgggcatggcctctggccacatcagggacttccagatcactgcctctggccagtatgggcagtgggccccaaagctggccaggctgcactattctgggagcatcaatgcttggagcaccaaggagcctttcagctggattaaggtggatctgctggcccccatgatcattcatggcatcaaaacccagggggctagacagaagttttctagcctgtacatcagccagttcatcatcatgtacagcctggatggcaagaagtggcagacttacaggggcaatagcactggcaccctgatggtgttttttggcaatgtggacagctctggcatcaagcacaacatctttaacccccccattattgccaggtatatcaggctgcatcccacccactattctattaggtctactctgagaatggagctgatgggctgtgacctgaacagctgtagcatgcccctggggatggagagcaaggctatctctgatgcccagatcactgccagctcttatttcaccaatatgtttgccacctggtctccctctaaggccaggctgcacctgcagggcaggagcaatgcttggaggccccaggtgaataaccccaaggagtggctgcaggtggacttccagaagaccatgaaggtgactggggtgactacccagggggtgaagtctctgctgactagcatgtatgtgaaggagttcctgatcagcagcagccaggatgggcatcagtggactctgttcttccagaatggcaaggtgaaggtcttccaggggaaccaggatagcttcactcctgtggtgaactctctggacccccccctgctgactaggtatctgaggatccacccccagagctgggtgcaccagattgccctgaggatggaggtgctgggctgtgaggcccaggacctgtattga

SEQ ID NO: 3 - DNA, 4374 bp, synthetic construct
  misc_feature 1..4374: note = Description of Artificial Sequence: FVIII Nucleic Acid
  source 1..4374: mol_type = other DNA
atgcagattgaactgtctacttgtttcttcctgtgcctgctgaggttttgcttctctgctactaggaggtactatctgggggctgtggagctgtcttgggactatatgcagtctgacctgggggagctgcctgtggatgctaggtttccccccagggtgcccaagagcttcccctttaacacctctgtggtgtataagaagactctgtttgtggagttcactgaccatctgttcaacattgccaagccaaggcccccctggatgggcctgctgggccccaccatccaggctgaggtgtatgacactgtggtgattactctgaagaacatggccagccatcctgtgagcctgcatgctgtgggggtgtcttactggaaggcctctgagggggctgagtatgatgaccagacctctcagagggagaaggaggatgacaaggtgttccctgggggctctcatacctatgtgtggcaggtcctgaaggagaatgggcccatggcctctgaccccctgtgcctgacctactcttatctgtctcatgtggacctggtgaaggacctgaactctggcctgattggggccctgctggtgtgcagggagggcagcctggctaaggagaagacccagactctgcacaagttcatcctgctgtttgctgtgtttgatgagggcaagagctggcactctgagaccaagaacagcctgatgcaggacagggatgctgcctctgctagggcctggcccaagatgcacactgtgaatgggtatgtgaacaggagcctgccaggcctgattggctgccataggaagtctgtgtattggcatgtgattgggatggggactacccctgaggtccacagcattttcctggaggggcatacctttctggtgaggaaccacaggcaggcctctctggagatctctcccattactttcctgactgcccagaccctgctgatggacctgggccagttcctgctgttctgccacatcagcagccaccagcatgatggcatggaggcctatgtgaaggtggatagctgccctgaggagccccagctgaggatgaaaaacaatgaggaggctgaggattatgatgatgacctgactgattctgagatggatgtggtgaggtttgatgatgataacagccccagcttcatccagattaggtctgtggccaagaagcatcccaagacctgggtgcactacattgctgctgaggaggaggattgggactatgctcctctggtgctggcccctgatgacaggagctacaagagccagtacctgaataatggcccccagaggattggcaggaagtataagaaggtgaggttcatggcctacactgatgagacctttaagaccagggaggccatccagcatgaatctgggatcctgggccccctgctgtatggggaggtgggggacaccctgctgattatctttaagaaccaggctagcaggccctacaacatttacccccatggcattactgatgtgaggcccctgtacagcaggaggctgcccaagggggtgaagcacctgaaggatttccccattctgcctggggagatctttaagtacaaatggactgtgactgtggaggatggccctactaagtctgatcccaggtgtctgaccagatactacagcagctttgtgaatatggagagggacctggcttctggcctgattggccccctgctgatctgctacaaggagtctgtggaccagaggggcaatcagattatgtctgacaagaggaatgtgatcctgttctctgtgtttgatgagaacagaagctggtacctgactgagaacatccagaggttcctgcccaaccctgctggggtgcagctggaggaccctgagttccaggctagcaatatcatgcacagcattaatggctatgtgtttgacagcctgcagctgtctgtgtgcctgcatgaggtggcctattggtacattctgagcattggggcccagactgatttcctgtctgtgttcttttctggctacaccttcaagcacaagatggtgtatgaggatactctgaccctgtttcccttctctggggagactgtgttcatgagcatggagaaccctggcctgtggatcctgggctgtcacaactctgacttcaggaacaggggcatgactgccctgctgaaggtgagctcttgtgataagaacactggggactactatgaggactcttatgaggacatctctgcctacctgctgagcaagaacaatgctattgagcccaggagcttctctcagaatccccctgtgctgaagaggcatcagagggagatcactaggactaccctgcagtctgaccaggaagagattgactatgatgacaccatctctgtggaaatgaagaaggaggactttgatatctatgatgaggatgaaaaccagagccccaggagcttccagaagaagaccaggcattacttcattgctgctgtggagaggctgtgggactatgggatgagctcttctccccatgtgctgaggaatagggctcagtctggctctgtcccacagttcaagaaggtggtgtttcaggagttcactgatggcagcttcactcagcccctgtacaggggggagctgaatgagcatctgggcctgctggggccctacatcagggctgaggtggaggataacattatggtgactttcaggaaccaggcctctaggccctacagcttctacagcagcctgatcagctatgaggaggaccagaggcagggggctgagcccaggaagaactttgtgaagcccaatgagactaagacctatttctggaaggtgcagcatcacatggctcccactaaagatgagtttgactgcaaggcctgggcctacttctctgatgtggatctggagaaggatgtgcattctgggctgattggccctctgctggtctgccatactaacaccctgaatcctgcccatggcaggcaggtgactgtgcaggagtttgccctgttctttaccatctttgatgagaccaagtcttggtacttcactgagaacatggagaggaactgcagggccccctgtaacatccagatggaggaccccacctttaaggagaactacaggttccatgccatcaatggctacatcatggacactctgcctggcctggtgatggcccaggaccagaggatcaggtggtacctgctgtctatgggctctaatgagaacattcattctatccacttctctggccatgtgtttactgtgaggaagaaggaggagtacaagatggccctgtacaatctgtaccctggggtgtttgaaactgtggagatgctgccctctaaggctggcatctggagggtggagtgcctgattggggaacacctgcatgctggcatgagcaccctgttcctggtctatagcaataagtgccagacccccctggggatggcctctgggcatatcagagacttccagatcactgcctctggccagtatggccagtgggcccccaagctggccaggctgcactactctggcagcattaatgcctggagcaccaaggagcccttctcttggatcaaggtggacctgctggctcccatgatcatccatgggatcaagacccagggggccaggcagaagttcagcagcctgtacatctctcagttcatcatcatgtactctctggatggcaagaagtggcagacctacaggggcaatagcactgggaccctgatggtgttctttgggaatgtggacagctctggcatcaagcacaatatcttcaacccccccatcattgccaggtacatcagactgcaccccactcattacagcatcaggagcactctgaggatggagctgatgggctgtgacctgaatagctgctctatgcccctgggcatggagagcaaggccatttctgatgcccagattactgcctcttcttacttcactaatatgtttgccacctggagccccagcaaggccaggctgcatctgcaggggaggagcaatgcctggaggccccaggtgaacaaccccaaggagtggctgcaggtggacttccagaagactatgaaggtgactggggtgaccactcagggggtgaagagcctgctgaccagcatgtatgtgaaggagttcctgatctcttctagccaggatgggcaccagtggaccctgtttttccagaatgggaaggtgaaggtgtttcagggcaatcaggacagctttactcctgtggtgaacagcctggacccccccctgctgactaggtacctgaggattcacccccagagctgggtgcaccagattgccctgaggatggaggtgctgggctgtgaggcccaggatctgtactga

SEQ ID NO: 4 - DNA, 4374 bp, synthetic construct
  misc_feature 1..4374: note = Description of Artificial Sequence: FVIII Nucleic Acid
  source 1..4374: mol_type = other DNA
atgcagattgagctgtctacctgcttctttctgtgcctgctgaggttctgtttctctgccactaggaggtattatctgggggctgtggagctgtcctgggactacatgcagtctgatctgggggagctgcctgtggatgccaggttccctcccagggtgcccaagtctttccctttcaatacctctgtggtgtacaagaagactctgtttgtggagtttactgatcacctgtttaacattgccaagcccaggcccccctggatggggctgctgggccccaccatccaggctgaggtgtatgacactgtggtgattactctgaagaatatggcttctcaccctgtgagcctgcatgctgtgggggtgagctactggaaggcctctgagggggctgagtatgatgaccagaccagccagagggagaaggaggatgacaaggtgttccctgggggcagccacacttatgtgtggcaggtgctgaaggagaatggcccaatggcctctgaccccctgtgcctgacctacagctatctgagccatgtggatctggtgaaggatctgaactctggcctgattggggccctgctggtgtgcagggagggctctctggccaaggagaagactcagactctgcacaagttcatcctgctgtttgctgtgtttgatgagggcaagagctggcactctgagaccaagaactctctgatgcaggatagggatgctgcttctgccagggcctggcccaagatgcacactgtgaatgggtatgtgaataggagcctgcctgggctgattgggtgtcacaggaagtctgtgtactggcatgtgattggcatgggcaccactcctgaggtgcacagcatctttctggagggccacacttttctggtgaggaatcacaggcaggccagcctggagatcagccccatcaccttcctgactgcccagaccctgctgatggatctgggccagttcctgctgttttgccatatcagcagccatcagcatgatgggatggaggcttatgtgaaggtggactcttgccctgaggagcctcagctgaggatgaagaataatgaagaggctgaggactatgatgatgatctgactgactctgagatggatgtggtgaggtttgatgatgacaacagccccagctttatccagattaggtctgtggccaagaagcaccccaagacctgggtgcattacattgctgctgaggaagaggattgggactatgcccccctggtgctggcccctgatgacaggagctacaagtctcagtacctgaacaatggccctcagaggattggcaggaagtacaagaaggtgaggttcatggcttacactgatgagaccttcaagaccagggaggccattcagcatgaatctgggatcctgggccccctgctgtatggggaggtgggggacaccctgctgattattttcaagaaccaggccagcaggccctacaacatttatcctcatggcattactgatgtgagacccctgtacagcaggaggctgcctaagggggtgaagcacctgaaggacttccccatcctgcctggggagatcttcaagtacaagtggactgtgactgtggaggatggccccactaagtctgaccccaggtgcctgactaggtactactccagctttgtgaacatggagagggacctggcctctggcctgattggccccctgctgatctgctacaaggagtctgtggatcagaggggcaaccagatcatgtctgacaagagaaatgtgatcctgttctctgtgtttgatgagaataggtcttggtacctgactgagaacatccagaggtttctgcctaatcctgctggggtgcagctggaggatcctgagttccaggcctctaacattatgcacagcatcaatgggtatgtgtttgacagcctgcagctgtctgtgtgcctgcatgaggtggcctactggtacatcctgagcattggggcccagactgactttctgtctgtgttcttctctggctacacctttaagcataagatggtgtatgaggacaccctgactctgttccccttctctggggagactgtgttcatgagcatggagaacccaggcctgtggatcctgggctgccacaactctgatttcaggaataggggcatgactgccctgctgaaggtgagcagctgtgataagaacactggggactattatgaggatagctatgaggacatctctgcctacctgctgagcaagaacaatgccattgagcccaggagcttcagccagaatcctcctgtgctgaagaggcaccagagggagatcaccaggaccaccctgcagtctgatcaggaggagattgactatgatgacactatctctgtggagatgaagaaggaggactttgacatctatgatgaggatgagaatcagagccccaggagcttccagaagaagactagacactactttattgctgctgtggagaggctgtgggactatggcatgagctcttctccccatgtgctgagaaacagggcccagtctggctctgtgccccagttcaagaaggtggtcttccaggagttcactgatggctctttcacccagcctctgtatagaggggagctgaatgagcacctgggcctgctgggcccttacatcagggctgaggtggaggacaatatcatggtgaccttcaggaaccaggctagcaggccctactctttctacagcagcctgatcagctatgaggaggaccagaggcagggggctgagcctaggaagaattttgtgaagcccaatgagaccaagacctacttctggaaggtgcagcaccacatggctcccactaaggatgagtttgactgcaaggcctgggcctacttttctgatgtggacctggagaaggatgtgcattctggcctgattggccccctgctggtctgccacaccaatactctgaaccctgctcatgggagacaggtgactgtgcaggagtttgccctgttcttcaccatctttgatgagaccaagtcctggtactttactgagaacatggagaggaattgcagggccccttgcaacatccagatggaggaccccaccttcaaggaaaattataggttccatgccatcaatggctacatcatggacaccctgcctggcctggtgatggcccaggaccagaggatcaggtggtatctgctgtctatgggctctaatgagaacatccacagcatccatttctctggccatgtgttcactgtgaggaagaaggaggagtataagatggctctgtacaacctgtaccctggggtctttgagactgtggagatgctgcccagcaaggctggcatttggagggtggagtgcctgattggggaacacctgcatgctgggatgagcaccctgttcctggtgtactctaacaagtgccagaccccactgggcatggcttctggccacatcagggatttccagattactgcctctggccagtatggccagtgggctcccaagctggctaggctgcactactctgggagcatcaatgcctggtctactaaggagcctttctcttggatcaaagtggacctgctggcccctatgatcatccatgggatcaagactcagggggccaggcagaagttcagcagcctgtacatctctcagttcatcattatgtacagcctggatggcaagaagtggcagacctacaggggcaacagcactggcaccctgatggtgttctttgggaatgtggacagctctgggattaagcacaacatctttaacccccccatcattgccaggtatatcaggctgcaccctacccactacagcattaggagcaccctgaggatggagctgatgggctgtgacctgaacagctgcagcatgcccctggggatggagagcaaggccatttctgatgctcagatcactgcttctagctacttcactaacatgtttgccacctggtctcccagcaaggctagactgcacctgcaggggaggagcaatgcctggaggccccaggtgaataatcccaaggagtggctgcaggtggatttccagaaaaccatgaaggtgactggggtgactacccagggggtgaagtctctgctgaccagcatgtatgtgaaggagttcctgatcagcagcagccaggatgggcatcagtggaccctgttctttcagaatgggaaggtgaaggtgtttcagggcaatcaggacagcttcacccctgtggtgaacagcctggacccccccctgctgaccaggtacctgaggatccacccccagagctgggtgcatcagattgccctgaggatggaggtgctgggctgtgaggcccaggacctgtactga

SEQ ID NO: 5 - DNA, 4374 bp, synthetic construct
  misc_feature 1..4374: note = Description of Artificial Sequence: FVIII Nucleic Acid
  source 1..4374: mol_type = other DNA
atgcagattgagctgtctacttgcttcttcctgtgcctgctgaggttctgcttctctgccactaggaggtattacctgggggctgtggagctgagctgggactatatgcagtctgacctgggggagctgcctgtggatgccaggtttcctcccagggtgcctaagagcttccccttcaacacctctgtggtgtacaagaagactctgtttgtggagtttactgatcatctgttcaacattgccaagcccaggcctccttggatggggctgctgggccccaccatccaggctgaggtgtatgacactgtggtgattaccctgaagaatatggccagccatcctgtgagcctgcatgctgtgggggtgagctattggaaggcctctgagggggctgagtatgatgatcagactagccagagggagaaggaggatgacaaggtgttccctggggggagccatacctatgtgtggcaggtgctgaaggagaatggccccatggcctctgaccctctgtgcctgacttatagctacctgagccatgtggatctggtgaaggacctgaactctggcctgattggggccctgctggtgtgcagggagggcagcctggccaaggagaagactcagaccctgcacaagttcatcctgctgtttgctgtgtttgatgaggggaagtcctggcactctgagactaagaacagcctgatgcaggatagggatgctgcttctgccagggcctggcctaagatgcacactgtgaatggctatgtgaataggagcctgcctggcctgattggctgccataggaagtctgtgtactggcatgtgattgggatgggcaccacccctgaggtgcactctattttcctggagggccatactttcctggtgaggaaccataggcaggccagcctggagatcagccccatcactttcctgactgcccagactctgctgatggacctgggccagttcctgctgttctgccacatcagcagccatcagcatgatggcatggaggcttatgtgaaggtggacagctgccctgaggagcctcagctgaggatgaagaataatgaggaggctgaggactatgatgatgacctgactgactctgagatggatgtggtgaggtttgatgatgacaactctccctctttcatccagatcaggtctgtggccaagaagcaccctaagacctgggtgcactacattgctgctgaggaggaggattgggactatgcccccctggtgctggccccagatgacaggagctacaagtcccagtacctgaacaatggcccccagaggattggcaggaagtacaagaaggtgaggttcatggcttatactgatgagactttcaagaccagggaggccatccagcatgagtctggcatcctgggccctctgctgtatggggaggtgggggacaccctgctgattatcttcaagaaccaggcttctaggccctacaatatctaccctcatggcatcactgatgtgaggcccctgtacagcaggaggctgcccaagggggtgaagcatctgaaggatttccccatcctgcctggggagatctttaagtataagtggactgtgactgtggaggatggccccactaagtctgaccccaggtgcctgaccaggtattacagcagctttgtgaacatggagagggatctggcttctgggctgattggccccctgctgatctgctacaaggagtctgtggaccagaggggcaaccagatcatgtctgacaagaggaatgtgatcctgttctctgtgtttgatgagaataggagctggtacctgactgagaacatccagaggtttctgcccaatcctgctggggtgcagctggaggatcctgagtttcaggcctctaatatcatgcacagcatcaatggctatgtgtttgactctctgcagctgtctgtgtgcctgcatgaggtggcctattggtacatcctgagcattggggcccagactgactttctgtctgtgtttttttctggctacaccttcaagcacaagatggtgtatgaggatactctgactctgttccctttttctggggagactgtgttcatgtctatggagaaccctgggctgtggattctgggctgccacaattctgacttcaggaacagaggcatgactgctctgctgaaggtgagcagctgtgacaagaacactggggactactatgaggactcttatgaggacatttctgcctacctgctgagcaagaacaatgccattgagcccagaagcttttctcagaacccccctgtgctgaagaggcaccagagggagatcaccaggaccaccctgcagtctgaccaggaggagattgactatgatgatactatttctgtggagatgaagaaggaggactttgacatctatgatgaggatgagaaccagagccccaggtctttccagaagaagactaggcactactttattgctgctgtggagaggctgtgggactatgggatgtctagctctcctcatgtgctgaggaacagggcccagtctggctctgtgccccagtttaaaaaggtggtgttccaggaattcactgatggcagctttacccagcctctgtacaggggggagctgaatgagcacctggggctgctggggccttacattagggctgaggtggaggacaacatcatggtgaccttcaggaatcaggccagcaggccctactctttctacagcagcctgatctcttatgaggaggaccagaggcagggggctgaacccaggaagaactttgtgaagcccaatgagaccaagacctacttctggaaggtgcagcaccacatggctcccaccaaggatgagtttgattgcaaggcctgggcttacttctctgatgtggatctggagaaggatgtgcactctgggctgattggccccctgctggtgtgccacaccaacactctgaaccctgcccatggcagacaggtgactgtgcaggagtttgccctgttcttcactatctttgatgagactaagagctggtacttcactgagaacatggagaggaattgcagggccccttgcaacatccagatggaggaccccacctttaaggagaactacaggtttcatgccattaatggctacatcatggacaccctgcctggcctggtgatggcccaggaccagaggatcaggtggtacctgctgtctatggggagcaatgagaacatccacagcattcacttctctggccatgtgttcactgtgaggaagaaggaggagtacaagatggccctgtacaacctgtaccctggggtgtttgagactgtggagatgctgcccagcaaggctgggatctggagggtggagtgcctgattggggagcacctgcatgctgggatgagcaccctgttcctggtgtatagcaacaagtgccagacccccctgggcatggcctctggccacatcagagactttcagattactgcctctggccagtatgggcagtgggcccccaagctggccaggctgcactattctggctctattaatgcctggagcactaaggagcccttcagctggattaaggtggacctgctggctcccatgatcatccatggcatcaagactcagggggccaggcagaagttctcttctctgtacatcagccagttcattatcatgtactccctggatggcaagaagtggcagacctataggggcaacagcactggcaccctgatggtgttctttgggaatgtggacagctctggcatcaagcataatatcttcaatccccccatcattgctaggtacatcaggctgcaccccacccactactctattaggtctaccctgaggatggagctgatgggctgtgacctgaacagctgcagcatgcctctgggcatggagagcaaagccatctctgatgcccagatcactgccagcagctactttaccaacatgtttgctacttggagccccagcaaggccaggctgcacctgcaggggaggtctaatgcctggaggccccaggtgaacaaccccaaggagtggctgcaggtggacttccagaagactatgaaggtgactggggtgaccacccagggggtgaagagcctgctgacctctatgtatgtgaaggagttcctgattagcagcagccaggatggccaccagtggaccctgtttttccagaatgggaaggtgaaggtgtttcaggggaaccaggacagcttcactcctgtggtgaactctctggacccccccctgctgaccaggtatctgaggatccaccctcagagctgggtgcaccagattgccctgaggatggaggtgctgggctgtgaggcccaggacctgtactga

SEQ ID NO: 6 - DNA, 4374 bp, synthetic construct
  misc_feature 1..4374: note = Description of Artificial Sequence: FVIII Nucleic Acid
  source 1..4374: mol_type = other DNA
atgcagattgagctgagcacctgcttcttcctgtgcctgctgaggttttgcttctctgccaccaggaggtactacctgggggctgtggagctgagctgggattacatgcagtctgacctgggggagctgcctgtggatgccaggttccctcccagggtgcccaagtctttccccttcaacacttctgtggtgtacaagaagaccctgtttgtggagtttactgaccacctgttcaacattgccaagcccaggcctccctggatgggcctgctgggccccaccattcaggctgaggtgtatgacactgtggtcatcaccctgaaaaatatggctagccaccctgtgtctctgcatgctgtgggggtgagctactggaaggcctctgagggggctgagtatgatgaccagactagccagagggagaaggaggatgacaaggtgttccctgggggcagccacacttatgtgtggcaggtgctgaaagagaatggccccatggcttctgatcccctgtgtctgacctatagctacctgagccatgtggatctggtgaaggacctgaactctggcctgattggggccctgctggtgtgcagggagggcagcctggctaaggagaagacccagaccctgcataagttcatcctgctgtttgctgtgtttgatgagggcaagagctggcactctgagactaagaacagcctgatgcaggatagggatgctgcttctgccagggcctggcccaagatgcacactgtgaatgggtatgtgaacaggagcctgcctggcctgattggctgccataggaagtctgtctattggcatgtgattggcatgggcactactcctgaggtgcacagcatctttctggagggccacaccttcctggtgaggaaccacaggcaggccagcctggagatctctcccatcactttcctgactgctcagaccctgctgatggacctgggccagttcctgctgttctgtcacatctctagccaccagcatgatggcatggaggcctatgtgaaggtggatagctgccctgaggaaccccagctgaggatgaagaacaatgaggaggctgaggattatgatgatgatctgactgattctgagatggatgtggtgaggtttgatgatgacaattctcctagcttcattcagatcagatctgtggccaaaaagcatcctaagacttgggtgcattatattgctgctgaggaggaggattgggattatgcccccctggtgctggctcctgatgataggagctacaagtctcagtacctgaataatgggccccagaggattggcaggaagtacaagaaggtgaggttcatggcctacactgatgagaccttcaagaccagggaggccattcagcatgagtctgggattctggggcccctgctgtatggggaggtgggggataccctgctgatcattttcaagaaccaggccagcaggccctacaacatctacccccatgggattactgatgtgaggcccctgtactctaggaggctgcctaagggggtgaagcacctgaaggattttcctatcctgcctggggaaatcttcaagtacaagtggactgtgactgtggaggatggccccactaagtctgatcccaggtgtctgaccaggtattatagctcttttgtgaacatggagagggatctggcctctgggctgattggccctctgctgatctgctacaaggagtctgtggaccagaggggcaaccagatcatgtctgacaagaggaatgtgatcctgttctctgtgtttgatgagaacaggagctggtatctgactgagaacatccagaggtttctgcccaatcctgctggggtgcagctggaggatcctgagttccaggctagcaacatcatgcacagcatcaatgggtatgtgtttgacagcctgcagctgtctgtgtgtctgcatgaggtggcctactggtatatcctgtctattggggcccagactgacttcctgtctgtgtttttttctgggtatacttttaagcacaagatggtgtatgaggacaccctgactctgttccccttctctggggagactgtgtttatgagcatggagaaccctggcctgtggatcctgggctgccacaattctgacttcaggaatagggggatgactgccctgctgaaggtgagcagctgtgataagaatactggggactactatgaggactcttatgaggacatttctgcctatctgctgtctaagaacaatgccattgaacccaggagcttctctcagaacccccctgtgctgaagaggcaccagagggaaatcaccagaactactctgcagtctgatcaggaggaaattgactatgatgacactatttctgtggagatgaagaaggaggactttgacatctatgatgaggatgagaaccagagcccaaggagcttccagaagaagactaggcactacttcattgctgctgtggagaggctgtgggactatggcatgagcagcagcccccatgtgctgagaaacagggcccagtctgggtctgtgccccagttcaagaaggtggtgttccaggagttcactgatgggagcttcacccagcccctgtataggggggagctgaatgagcacctgggcctgctgggcccctatattagggctgaggtggaggacaacatcatggtgaccttcaggaatcaggcctctaggccctacagcttctacagcagcctgattagctatgaggaggatcagaggcagggggctgaacccaggaagaactttgtgaagcccaatgagaccaagacctatttctggaaggtgcagcatcacatggcccccaccaaggatgagtttgactgcaaggcctgggcctacttctctgatgtggatctggagaaggatgtgcactctggcctgattggccccctgctggtgtgccacaccaacaccctgaaccctgctcatggcaggcaggtgactgtgcaggagtttgccctgttcttcaccatctttgatgagactaagtcttggtacttcactgagaatatggagaggaattgcagggccccctgcaatattcagatggaagaccccaccttcaaggagaattacaggttccatgccattaatggctacatcatggataccctgcctggcctggtgatggcccaggatcagaggatcaggtggtacctgctgagcatgggcagcaatgagaacatccactctatccacttctctggccatgtgtttactgtgaggaagaaggaggagtataagatggccctgtacaacctgtaccctggggtctttgagactgtggagatgctgccttctaaggctggcatttggagggtggagtgcctgattggggaacacctgcatgctggcatgtctaccctgttcctggtgtacagcaataagtgccagacccccctgggcatggcctctgggcatatcagggatttccagatcactgcctctggccagtatggccagtgggccccaaagctggctaggctgcactactctgggagcatcaatgcctggagcactaaggagcccttcagctggatcaaggtggacctgctggcccccatgattatccatgggattaagactcagggggccaggcagaagttcagcagcctgtacatcagccagttcattatcatgtacagcctggatggcaagaagtggcagacctataggggcaactctactgggaccctgatggtgttctttgggaatgtggatagctctgggatcaagcacaatatcttcaacccccccatcattgccaggtatatcaggctgcaccccacccactacagcattaggtctaccctgaggatggagctgatgggctgtgatctgaacagctgtagcatgcctctgggcatggagtctaaggccatttctgatgcccagattactgctagcagctacttcaccaacatgtttgccacctggtctcccagcaaggccaggctgcatctgcagggcaggtctaatgcttggaggccccaggtgaacaacccaaaggagtggctgcaggtggatttccagaagactatgaaggtgactggggtgaccactcagggggtgaagtctctgctgacctctatgtatgtgaaggagttcctgatctctagcagccaggatggccatcagtggaccctgttcttccagaatggcaaggtgaaagtgttccagggcaatcaggatagcttcactccagtggtgaacagcctggatccccctctgctgactaggtacctgaggatccacccccagagctgggtgcaccagattgccctgaggatggaggtgctgggctgtgaggcccaggacctgtactga

SEQ ID NO: 7 - DNA, 4374 bp, synthetic construct
  misc_feature 1..4374: note = Description of Artificial Sequence: FVIII Nucleic Acid
  source 1..4374: mol_type = other DNA
atgcagattgagctgagcacctgcttcttcctgtgtctgctgaggttctgcttctctgccaccaggaggtattacctgggggctgtggagctgagctgggactatatgcagtctgacctgggggagctgcctgtggatgctaggttcccccccagggtgcccaagagcttcccctttaacacttctgtggtgtacaagaagaccctgtttgtggagttcactgaccacctgttcaacattgccaagcccaggcccccctggatggggctgctggggcccaccatccaggctgaggtgtatgacactgtggtgatcaccctgaagaacatggccagccaccctgtgagcctgcatgctgtgggggtgagctactggaaggcttctgagggggctgagtatgatgaccagactagccagagggagaaggaggatgacaaggtgtttcctgggggcagccatacctatgtgtggcaggtgctgaaggagaatggccccatggcctctgaccccctgtgcctgacctacagctacctgtctcatgtggacctggtgaaggacctgaactctggcctgattggggctctgctggtgtgtagggagggcagcctggctaaggaaaagacccagaccctgcataagtttatcctgctgtttgctgtgtttgatgagggcaagagctggcactctgagaccaagaacagcctgatgcaggatagggatgctgcctctgccagggcttggcctaagatgcacactgtgaatgggtatgtgaataggagcctgcctggcctgattggctgccacaggaagtctgtgtactggcatgtgattgggatgggcaccacccctgaggtccatagcatcttcctggagggccacactttcctggtgaggaaccacagacaggcctctctggagatctctcccatcaccttcctgactgctcagactctgctgatggacctgggccagttcctgctgttttgccatattagcagccaccagcatgatgggatggaggcctatgtgaaggtggatagctgccctgaggagcctcagctgaggatgaagaacaatgaggaggctgaagactatgatgatgacctgactgattctgagatggatgtggtgaggtttgatgatgacaatagccccagcttcattcagatcaggtctgtggccaagaaacaccccaagacctgggtgcactacattgctgctgaggaagaggactgggactatgctcccctggtgctggcccctgatgataggtcttataagagccagtacctgaacaatgggccccagaggattggcaggaagtacaagaaggtgaggttcatggcctacactgatgaaaccttcaaaaccagggaggccattcagcatgagtctggcatcctgggccctctgctgtatggggaggtgggggacaccctgctgatcatcttcaagaaccaggccagcaggccctacaacatctatcctcatggcatcactgatgtgaggcccctgtacagcaggaggctgcccaagggggtgaagcacctgaaagacttccccatcctgcctggggagatctttaagtataagtggactgtgactgtggaggatggccctaccaagtctgaccccaggtgtctgaccaggtactattctagctttgtgaacatggagagggacctggcctctggcctgattgggcccctgctgatctgctacaaggagtctgtggaccagaggggcaaccagatcatgtctgacaagaggaatgtgatcctgttttctgtgtttgatgagaataggagctggtacctgactgagaacatccagaggtttctgcccaatcctgctggggtgcagctggaggatcctgagttccaggccagcaatatcatgcatagcatcaatggctatgtgtttgacagcctgcagctgtctgtgtgcctgcatgaggtggcctactggtacatcctgagcattggggcccagactgactttctgtctgtgttcttttctggctataccttcaagcacaagatggtgtatgaggataccctgaccctgttccccttctctggggagactgtgttcatgagcatggagaatcctgggctgtggatcctggggtgccacaactctgattttaggaacagggggatgactgccctgctgaaggtgtctagctgtgataagaacactggggactactatgaggacagctatgaggacatttctgcttatctgctgtctaagaataatgccattgagcccagaagcttcagccagaatccccctgtgctgaagagacatcagagggagatcaccagaactaccctgcagtctgatcaggaggagattgactatgatgacactatctctgtggagatgaagaaggaggactttgacatctatgatgaggatgagaatcagtctcccaggagctttcagaagaagaccagacattacttcattgctgctgtggagaggctgtgggactatggcatgagctctagccctcatgtgctgaggaacagggcccagtctggctctgtgccccagttcaagaaggtggtgttccaggaattcactgatggcagcttcacccagcccctgtacaggggggagctgaatgagcacctgggcctgctggggccttatatcagggctgaggtggaggataatattatggtgactttcaggaaccaggccagcaggccctactctttctatagcagcctgatctcttatgaggaggatcagaggcagggggctgagcctaggaagaactttgtgaagcccaatgagactaagacctacttctggaaggtccagcaccacatggcccctaccaaggatgagtttgactgcaaggcctgggcctatttctctgatgtggatctggagaaggatgtccattctgggctgattggccccctgctggtgtgccacactaacactctgaatcctgcccatggcaggcaggtgactgtccaggagtttgccctgttcttcactatctttgatgagaccaagagctggtactttactgagaacatggagaggaactgcagagctccttgcaatattcagatggaggaccccaccttcaaggagaattacaggttccatgccattaatgggtacatcatggacaccctgcctggcctggtgatggctcaggaccagaggatcaggtggtacctgctgagcatgggctctaatgagaatatccacagcatccacttctctgggcatgtgttcactgtgaggaagaaggaggagtacaagatggctctgtataatctgtaccctggggtgtttgaaactgtggagatgctgccctctaaggctggcatctggagggtggagtgcctgattggggagcacctgcatgctggcatgagcaccctgttcctggtgtacagcaacaagtgccagacccccctgggcatggcctctggccacatcagggacttccagatcactgcctctggccagtatggccagtgggcccccaagctggccaggctgcactattctggcagcatcaatgcctggagcaccaaggagcccttcagctggatcaaggtggacctgctggcccccatgatcattcatggcatcaagacccagggggccaggcagaagttcagctctctgtacatctctcagttcatcatcatgtactctctggatgggaagaagtggcagacctacaggggcaacagcactggcaccctgatggtgttctttgggaatgtggactcttctggcatcaagcacaacatcttcaatccccccatcattgctaggtatattaggctgcatcccacccactacagcatcaggtctaccctgaggatggagctgatgggctgtgacctgaactcttgcagcatgcccctgggcatggagtctaaggccatctctgatgcccagattactgccagcagctacttcaccaacatgtttgccacctggagcccctctaaggccaggctgcatctgcaggggaggagcaatgcctggaggcctcaggtgaacaaccccaaggagtggctgcaggtggatttccagaagaccatgaaggtgactggggtgaccacccagggggtcaagagcctgctgaccagcatgtatgtgaaggagttcctgatcagcagcagccaggatggccaccagtggactctgttctttcagaatgggaaggtgaaggtgtttcagggcaatcaggactctttcacccctgtggtgaacagcctggacccccccctgctgaccagatacctgaggatccacccccagtcttgggtgcatcagattgccctgaggatggaggtgctgggctgtgaggctcaggatctgtactga

SEQ ID NO: 8 - DNA, 4374 bp, synthetic construct
  misc_feature 1..4374: note = Description of Artificial Sequence: FVIII Nucleic Acid
  source 1..4374: mol_type = other DNA
atgcagattgagctgagcacttgcttttttctgtgcctgctgaggttttgtttttctgccaccaggaggtactacctgggggctgtggagctgagctgggactatatgcagtctgatctgggggagctgcctgtggatgccaggttcccccccagggtgcccaagtcttttcccttcaacacctctgtggtgtataagaagaccctgtttgtggagttcactgaccacctgttcaacattgctaagcctaggcccccctggatgggcctgctgggccctaccattcaggctgaggtgtatgacactgtggtgatcaccctgaagaacatggccagccatcctgtgagcctgcatgctgtgggggtctcttactggaaggcctctgagggggctgagtatgatgaccagaccagccagagagagaaggaggatgacaaggtcttccctgggggctctcacacctatgtgtggcaggtgctgaaggaaaatggccccatggcctctgaccccctgtgcctgacctacagctatctgagccatgtggatctggtgaaggacctgaattctggcctgattggggccctgctggtgtgcagggagggcagcctggccaaggagaagacccagaccctgcacaagtttatcctgctgtttgctgtgtttgatgagggcaagtcttggcactctgagactaagaacagcctgatgcaggacagggatgctgcctctgccagggcctggcccaagatgcacactgtgaatggctatgtgaacaggagcctgcctgggctgattggctgccacaggaagtctgtgtactggcatgtgattggcatgggcaccacccctgaggtgcacagcatcttcctggaaggccacactttcctggtgaggaaccataggcaggccagcctggagatcagccctatcaccttcctgactgcccagaccctgctgatggatctggggcagttcctgctgttctgccacatctctagccaccagcatgatgggatggaggcctatgtgaaggtggacagctgcccagaggagcctcagctgaggatgaaaaacaatgaagaggctgaggattatgatgatgatctgactgactctgagatggatgtggtgagatttgatgatgacaatagccctagctttattcagatcaggtctgtggctaagaagcaccccaagacctgggtgcattacattgctgctgaggaggaggactgggattatgctcctctggtgctggcccctgatgataggagctacaagagccagtacctgaataatggccctcagaggattggcaggaagtacaagaaggtgaggttcatggcttacactgatgagaccttcaagactagggaggccatccagcatgagtctgggatcctggggcccctgctgtatggggaggtgggggacaccctgctgatcatcttcaagaaccaggctagcaggccttacaacatctatccccatgggatcactgatgtgagacctctgtacagcaggaggctgcccaagggggtcaagcatctgaaagacttccccatcctgcctggggagatctttaagtataagtggactgtgactgtggaggatgggcccaccaagtctgaccccaggtgcctgaccaggtattacagcagctttgtgaacatggagagggatctggcctctgggctgattggccccctgctgatctgttacaaggaatctgtggatcagaggggcaatcagatcatgtctgacaagaggaatgtgatcctgttctctgtgtttgatgagaataggtcttggtacctgactgaaaacatccagaggttcctgcccaaccctgctggggtccagctggaggatcctgagttccaggctagcaacatcatgcacagcatcaatgggtatgtgtttgatagcctgcagctgtctgtgtgcctgcatgaggtggcctactggtacatcctgtctattggggcccagactgacttcctgtctgtgttcttttctggctacaccttcaagcacaagatggtgtatgaggacaccctgaccctgttccccttctctggggagactgtctttatgagcatggagaaccctgggctgtggatcctgggctgccacaactctgatttcaggaataggggcatgactgctctgctgaaggtgagctcttgtgacaagaacactggggattactatgaggacagctatgaggacatttctgcctacctgctgagcaagaacaatgccattgagcctaggagctttagccagaatcctcctgtcctgaagaggcaccagagggagatcaccaggaccaccctgcagtctgaccaggaggagattgactatgatgataccatctctgtggagatgaagaaggaggactttgacatctatgatgaggatgagaatcagtctcccaggagcttccagaagaagaccaggcactatttcattgctgctgtggagaggctgtgggactatggcatgagcagctctcctcatgtgctgaggaatagggctcagtctggctctgtgccccagttcaagaaagtggtgtttcaggagttcactgatggctctttcacccagcctctgtataggggggagctgaatgagcacctggggctgctgggcccctatatcagggctgaggtggaggataacatcatggtgaccttcaggaaccaggcctctaggccctacagcttctatagcagcctgatcagctatgaggaggaccagaggcagggggctgagcccaggaagaactttgtgaagcccaatgagaccaagacttacttctggaaggtgcagcatcacatggcccccaccaaggatgagtttgactgtaaggcctgggcctacttctctgatgtggatctggagaaggatgtgcactctggcctgattggccccctgctggtgtgccataccaatactctgaaccctgctcatggcaggcaggtgactgtgcaggagtttgctctgttcttcactatctttgatgagaccaagtcttggtatttcactgagaatatggagaggaactgcagggccccctgcaacatccagatggaggaccccacctttaaggagaactataggtttcatgccatcaatggctacatcatggacaccctgcctggcctggtgatggcccaggatcagaggatcaggtggtacctgctgagcatggggtctaatgagaacatccacagcatccacttctctggccatgtgtttactgtgagaaagaaggaggagtacaagatggctctgtacaatctgtaccctggggtctttgagactgtggagatgctgcctagcaaggctgggatctggagggtggagtgcctgattggggaacatctgcatgctgggatgtctactctgttcctggtgtacagcaacaagtgccagacccccctgggcatggcttctggccatatcagggactttcagattactgcctctgggcagtatggccagtgggcccccaagctggctaggctgcattattctggcagcatcaatgcctggtctactaaggagcccttcagctggatcaaggtggatctgctggcccccatgatcatccatggcatcaagacccagggggccaggcagaagtttagctctctgtacattagccagttcatcatcatgtacagcctggatgggaagaagtggcagacctacaggggcaattctactggcaccctgatggtgttctttggcaatgtggacagctctggcatcaagcacaacatctttaacccccctatcattgctaggtacatcaggctgcatcccacccattacagcatcaggagcaccctgaggatggagctgatgggctgtgacctgaactcttgcagcatgcccctgggcatggagagcaaggccatttctgatgcccagattactgccagcagctacttcactaacatgtttgccacctggtctcccagcaaggccaggctgcacctgcagggcaggagcaatgcctggaggccccaggtgaacaaccccaaggagtggctgcaggtggatttccagaagaccatgaaggtgactggggtgaccacccagggggtgaagagcctgctgactagcatgtatgtgaaggagttcctgatcagctctagccaggatggccaccagtggactctgtttttccagaatggcaaggtgaaggtgttccagggcaaccaggactctttcactcctgtggtgaacagcctggacccccccctgctgaccaggtatctgaggattcacccccagtcttgggtgcatcagattgccctgaggatggaggtgctgggctgtgaggcccaggatctgtactga

SEQ ID NO: 9 - DNA, 4374 bp, synthetic construct
  misc_feature 1..4374: note = Description of Artificial Sequence: FVIII Nucleic Acid
  source 1..4374: mol_type = other DNA
atgcagattgagctgagcacctgcttcttcctgtgtctgctgagattttgcttttctgccactaggaggtattacctgggggctgtggagctgtcttgggactacatgcagtctgatctgggggagctgcctgtggatgccaggttcccacctagggtgcctaagagctttcccttcaatacctctgtggtgtacaagaagaccctgtttgtggagttcactgaccacctgttcaacattgccaagcctaggcccccctggatgggcctgctgggccctaccatccaggctgaagtgtatgacactgtggtgatcaccctgaagaacatggccagccaccctgtgagcctgcatgctgtgggggtgtcttactggaaggcctctgagggggctgagtatgatgatcagaccagccagagggagaaggaagatgacaaggtgttccctgggggcagccacacctatgtctggcaggtgctgaaggagaatggccccatggcctctgatcccctgtgcctgacctactcttacctgagccatgtggacctggtgaaggatctgaattctggcctgattggggccctgctggtgtgcagggagggcagcctggccaaggagaagacccagaccctgcataagttcatcctgctgtttgctgtgtttgatgaagggaagagctggcactctgagactaagaacagcctgatgcaggacagggatgctgcttctgccagggcctggcccaagatgcacactgtgaatggctatgtgaatagaagcctgcctggcctgattgggtgccacaggaagtctgtgtactggcatgtgattgggatgggcactacccctgaggtgcatagcatcttcctggaaggccataccttcctggtgaggaatcataggcaggcttctctggaaatttctcccatcactttcctgactgctcagaccctgctgatggacctgggccagttcctgctgttctgccacatcagctctcaccagcatgatgggatggaggcctatgtgaaggtggacagctgtcctgaggagccccagctgaggatgaagaacaatgaggaggctgaggactatgatgatgacctgactgactctgagatggatgtggtcaggtttgatgatgacaatagcccctctttcatccagatcaggtctgtggccaagaagcaccccaagacttgggtgcactacattgctgctgaggaggaggattgggattatgcccctctggtgctggcccctgatgacaggagctataagtctcagtacctgaataatggcccccagaggattgggaggaagtataagaaggtgaggtttatggcctacactgatgagaccttcaagaccagggaggccatccagcatgagtctggcatcctgggccccctgctgtatggggaggtgggggataccctgctgatcatcttcaagaaccaggcctctaggccctacaatatctaccctcatggcatcactgatgtgagacccctgtatagcaggaggctgcctaagggggtgaagcacctgaaggacttccccatcctgcctggggagatcttcaagtataagtggactgtgactgtggaggatggccccaccaagtctgaccccaggtgcctgaccaggtattacagctcttttgtgaacatggagagggatctggcctctgggctgattggcccactgctgatctgctacaaggagtctgtggatcagaggggcaatcagatcatgtctgacaagaggaatgtgatcctgttttctgtgtttgatgaaaataggtcttggtatctgactgagaacatccagaggtttctgcccaatcctgctggggtgcagctggaggatcctgagtttcaggcctctaatatcatgcattctatcaatggctatgtgtttgacagcctgcagctgtctgtgtgcctgcatgaggtggcctactggtacatcctgagcattggggctcagactgacttcctgtctgtgttcttttctggctatactttcaagcacaagatggtgtatgaggacactctgaccctgttccccttctctggggagactgtgttcatgtctatggaaaatcctgggctgtggattctgggctgccacaattctgacttcaggaatagggggatgactgccctgctgaaggtgtctagctgtgataagaacactggggattactatgaggactcttatgaagatatctctgcctatctgctgagcaagaacaatgccattgagcccaggagcttcagccagaacccccctgtgctgaagaggcaccagagggagatcaccaggaccactctgcagtctgatcaggaggagattgactatgatgacactatctctgtggagatgaagaaggaggattttgacatttatgatgaggatgagaaccagtctcccaggagcttccagaagaagaccaggcattactttattgctgctgtggagaggctgtgggactatgggatgagcagctctcctcatgtgctgaggaacagggcccagtctgggtctgtgccccagttcaagaaggtggtgttccaggagttcactgatgggagcttcacccagcccctgtataggggggagctgaatgagcacctgggcctgctgggcccctacatcagggctgaggtggaggataatatcatggtgaccttcaggaaccaggctagcaggccttacagcttttacagcagcctgatctcttatgaagaagaccagaggcagggggctgagcccaggaagaattttgtgaagcctaatgagaccaagacttatttttggaaggtgcagcatcacatggctcctaccaaggatgagtttgactgcaaggcctgggcctacttttctgatgtggatctggagaaggatgtgcactctggcctgattggccctctgctggtgtgccatactaacactctgaaccctgcccatgggaggcaggtgactgtgcaggagtttgccctgttcttcactatttttgatgagaccaagtcttggtatttcactgagaacatggagaggaactgcagggctccctgcaacatccagatggaagaccccaccttcaaggagaactataggttccatgccatcaatgggtacatcatggataccctgcctggcctggtgatggcccaggatcagaggattaggtggtatctgctgagcatgggctctaatgagaacatccacagcatccatttctctggccatgtgttcactgtgaggaagaaggaggagtacaagatggctctgtacaacctgtatcctggggtgtttgagactgtggagatgctgcccagcaaggctggcatctggagggtggaatgcctgattggggagcacctgcatgctggcatgagcactctgttcctggtgtatagcaacaagtgccagacccccctgggcatggcctctggccatatcagggatttccagatcactgcttctggccagtatggccagtgggcccccaagctggccaggctgcactattctggcagcatcaatgcctggagcactaaggagcctttttcttggatcaaggtggacctgctggcccctatgattattcatggcatcaagacccagggggccaggcagaagttctctagcctgtacatctctcagttcatcattatgtatagcctggatggcaagaagtggcagacctacaggggcaatagcactggcaccctgatggtgttttttgggaatgtggactcttctgggatcaagcacaacatctttaacccccccatcattgccaggtatattaggctgcaccccacccactacagcatcaggagcaccctgaggatggagctgatgggctgtgatctgaattcttgctctatgcccctgggcatggagagcaaggccatctctgatgcccagatcactgccagctcttacttcaccaacatgtttgccacctggtctcctagcaaggccaggctgcatctgcagggcaggagcaatgcctggaggccccaggtgaacaaccccaaggagtggctgcaggtggacttccagaagaccatgaaggtgactggggtgaccactcagggggtgaagagcctgctgacctctatgtatgtgaaggagttcctgatcagcagcagccaggatggccaccagtggactctgttcttccagaatgggaaggtgaaggtgttccagggcaaccaggatagctttacccctgtggtgaacagcctggaccctcctctgctgaccagatacctgaggatccatcctcagagctgggtgcaccagattgccctgaggatggaggtgctgggctgtgaggcccaggatctgtactga

SEQ ID NO: 10 - DNA, 4374 bp, synthetic construct
  misc_feature 1..4374: note = Description of Artificial Sequence: FVIII Nucleic Acid
  source 1..4374: mol_type = other DNA
atgcagattgagctgagcacttgcttcttcctgtgcctgctgaggttctgcttttctgctactaggaggtactacctgggggctgtggagctgagctgggattacatgcagtctgacctgggggagctgccagtggatgccaggttcccccccagggtgcccaagtcttttcctttcaacacctctgtggtgtacaagaagaccctgtttgtggagttcactgaccacctgttcaacattgccaagcccaggcccccctggatggggctgctggggcccaccatccaggctgaggtgtatgacactgtggtgattaccctgaagaacatggctagccaccctgtgagcctgcatgctgtgggggtgagctattggaaggcctctgagggggctgagtatgatgatcagaccagccagagggaaaaggaggatgacaaggtgttccctgggggcagccatacttatgtgtggcaggtgctgaaggagaatgggcccatggcctctgaccccctgtgcctgacttacagctatctgagccatgtggacctggtgaaggatctgaactctggcctgattggggctctgctggtgtgcagggagggcagcctggctaaggagaagactcagactctgcataagttcatcctgctgtttgctgtgtttgatgaaggcaagagctggcactctgagaccaagaactctctgatgcaggatagggatgctgcctctgccagggcttggcccaagatgcacactgtgaatggctatgtgaacaggagcctgcctggcctgattgggtgccacaggaagtctgtgtactggcatgtgattggcatgggcaccacccctgaggtgcacagcattttcctggagggccacaccttcctggtgaggaatcacaggcaggccagcctggagatcagccccatcaccttcctgactgcccagaccctgctgatggacctggggcagtttctgctgttctgccacatcagcagccatcagcatgatggcatggaggcctatgtgaaggtggactcttgccctgaggagccccagctgaggatgaagaacaatgaggaggctgaggattatgatgatgacctgactgactctgagatggatgtggtgaggtttgatgatgacaatagccccagcttcatccagattaggtctgtggccaagaagcaccctaagacctgggtgcactacattgctgctgaggaggaggattgggattatgcccccctggtgctggctcctgatgacaggtcttataagagccagtacctgaacaatgggccccagaggattggcaggaagtacaagaaggtgaggttcatggcttacactgatgagaccttcaagactagggaggccatccagcatgagtctggcatcctgggccccctgctgtatggggaggtgggggataccctgctgatcatcttcaagaaccaggccagcaggccctacaacatttaccctcatggcatcactgatgtgaggcccctgtacagcaggagactgcccaagggggtgaagcacctgaaggattttcccattctgcctggggagatcttcaagtacaagtggactgtgactgtggaggatggccccaccaagtctgatcccaggtgcctgactaggtactactcttcttttgtgaatatggagagggatctggcctctggcctgattggccccctgctgatctgctacaaggagtctgtggaccagaggggcaaccagatcatgtctgacaagaggaatgtgatcctgttctctgtgtttgatgagaataggagctggtacctgactgagaatatccagaggttcctgcctaatcctgctggggtccagctggaggatcctgagttccaggctagcaacattatgcacagcatcaatggctatgtgtttgattctctgcagctgtctgtgtgcctgcatgaggtggcttactggtacatcctgtctattggggcccagactgatttcctgtctgtgttcttctctggctacactttcaagcataagatggtgtatgaggataccctgaccctgttccccttctctggggagactgtgttcatgtctatggagaaccctggcctgtggatcctgggctgtcataactctgacttcagaaacaggggcatgactgccctgctgaaggtgagcagctgtgacaagaacactggggactactatgaggacagctatgaggatatctctgcttatctgctgagcaagaataatgccattgagcccaggagcttcagccagaacccccctgtgctgaagaggcaccagagggagatcactaggactaccctgcagtctgatcaggaggagattgactatgatgacaccatctctgtggagatgaagaaggaggactttgacatctatgatgaggatgagaaccagtcccccaggtctttccagaagaagaccaggcactacttcattgctgctgtggagaggctgtgggactatggcatgagctctagcccccatgtgctgaggaacagggctcagtctggctctgtgccccagttcaagaaggtggtcttccaggagttcactgatggctcttttacccagcctctgtacagaggggagctgaatgagcacctgggcctgctgggcccctacatcagggctgaggtggaggataatatcatggtgaccttcagaaaccaggcctctaggccctacagcttctacagcagcctgatctcttatgaggaggatcagaggcagggggctgagcccaggaagaactttgtgaagcccaatgagaccaagacctacttctggaaggtgcagcaccatatggcccctactaaggatgagtttgactgcaaggcctgggcttatttttctgatgtggacctggagaaggatgtgcactctgggctgattggccccctgctggtgtgccacaccaacaccctgaaccctgcccatggcaggcaggtgactgtgcaggagtttgccctgttcttcactatctttgatgagaccaagagctggtacttcactgagaacatggagagaaattgtagggctccctgcaatatccagatggaggaccccaccttcaaagaaaattacagattccatgccatcaatgggtacatcatggataccctgcctgggctggtgatggctcaggaccagaggatcaggtggtacctgctgagcatggggtctaatgagaacatccactctatccatttctctggccatgtgttcactgtgagaaagaaggaggagtataagatggctctgtacaacctgtacccaggggtgtttgagactgtggaaatgctgcccagcaaagctgggatctggagggtggagtgcctgattggggagcacctgcatgctggcatgtctaccctgttcctggtgtacagcaacaagtgccagactcccctgggcatggcctctgggcacatcagggattttcagatcactgcctctggccagtatggccagtgggcccccaagctggccaggctgcactactctggcagcattaatgcttggagcactaaggagcccttcagctggatcaaggtggatctgctggcccccatgatcatccatggcatcaagacccagggggccaggcagaagttctctagcctgtacatttctcagttcatcatcatgtacagcctggatgggaagaagtggcagacctacagggggaacagcactgggaccctgatggtgttctttggcaatgtggatagctctggcatcaagcacaatatcttcaatccccccattattgccaggtacattaggctgcatcctactcactactctattaggagcaccctgaggatggagctgatggggtgtgacctgaacagctgttctatgcccctgggcatggagtctaaggctatctctgatgcccagatcactgccagcagctacttcactaatatgtttgccacctggagccctagcaaggccagactgcacctgcagggcaggagcaatgcctggaggccccaggtgaacaaccccaaggagtggctgcaggtggacttccagaagaccatgaaggtgactggggtgaccactcagggggtgaagagcctgctgaccagcatgtatgtgaaggagttcctgatcagcagcagccaggatggccaccagtggaccctgttcttccagaatgggaaggtgaaggtgttccagggcaaccaggactctttcacccctgtggtgaacagcctggatcctcccctgctgaccaggtacctgaggatccacccccagagctgggtgcaccagattgctctgaggatggaagtgctgggctgtgaggcccaggatctgtactga

SEQ ID NO: 11 - DNA, 4374 bp, synthetic construct
  misc_feature 1..4374: note = Description of Artificial Sequence: FVIII Nucleic Acid
  source 1..4374: mol_type = other DNA
atgcagattgagctgagcacctgcttcttcctgtgcctgctgaggttttgcttctctgctaccaggaggtactacctgggggctgtggagctgagctgggactatatgcagtctgacctgggggagctgcctgtggatgctaggttccctcccagggtgcccaagagcttcccctttaatacctctgtggtgtacaagaaaaccctgtttgtggagttcactgaccatctgttcaacattgccaagcccaggcccccttggatgggcctgctgggccccaccattcaggctgaggtgtatgacactgtggtcattaccctgaagaacatggcttctcaccctgtgagcctgcatgctgtgggggtgagctactggaaggcctctgagggggctgagtatgatgaccagaccagccagagggagaaggaggatgataaggtgttccctgggggcagccacacctatgtgtggcaggtgctgaaggagaatggccccatggcctctgatcccctgtgcctgacctactcttatctgtctcatgtggacctggtgaaggacctgaactctggcctgattggggctctgctggtgtgcagggagggctctctggccaaggagaagacccagaccctgcacaagtttattctgctgtttgctgtctttgatgagggcaagagctggcattctgagaccaagaacagcctgatgcaggacagggatgctgcctctgccagggcctggcccaaaatgcacactgtgaatggctatgtgaacaggagcctgcctggcctgattggctgccacaggaagtctgtgtactggcatgtgattggcatgggcaccacccctgaggtgcacagcatcttcctggagggccacacctttctggtgaggaatcacaggcaggccagcctggagattagccccatcaccttcctgactgcccagaccctgctgatggacctgggccagttcctgctgttctgccacatcagcagccaccagcatgatggcatggaggcctatgtgaaggtggatagctgccctgaggagccccagctgaggatgaaaaacaatgaggaggctgaggattatgatgatgacctgactgactctgagatggatgtggtgaggtttgatgatgacaatagccccagctttattcagattaggtctgtggctaagaagcaccccaagacttgggtgcactacattgctgctgaggaggaggattgggactatgcccctctggtcctggcccctgatgataggtcttacaagagccagtatctgaacaatggcccccagaggattggcaggaagtacaagaaggtgaggttcatggcctacactgatgagacctttaagaccagggaggccattcagcatgagtctgggatcctgggccccctgctgtatggggaggtgggggacactctgctgatcatcttcaagaaccaggccagcaggccttataacatctaccctcatgggatcactgatgtgaggcccctgtactctagaaggctgcccaagggggtcaagcacctgaaggattttcccatcctgcctggggagattttcaagtacaagtggactgtgactgtggaggatggccccaccaagtctgaccctaggtgcctgaccaggtactacagctcttttgtgaacatggagagggacctggcctctggcctgattggccctctgctgatttgctacaaggagtctgtggaccagaggggcaaccagatcatgtctgacaagaggaatgtgatcctgttttctgtgtttgatgagaacaggtcttggtacctgactgagaacatccagaggttcctgcctaacccagctggggtgcagctggaggatcctgagttccaggccagcaatattatgcatagcattaatggctatgtgtttgatagcctgcagctgtctgtgtgcctgcatgaggtggcctactggtacatcctgagcattggggcccagactgactttctgtctgtgttcttctctggctacaccttcaagcataagatggtgtatgaggacaccctgactctgttccctttttctggggagactgtgtttatgagcatggagaatcctggcctgtggatcctgggctgccataattctgacttcaggaacaggggcatgactgccctgctgaaagtgagcagctgtgacaagaatactggggactactatgaagacagctatgaggacatctctgcctacctgctgagcaagaacaatgccattgagcccaggagcttcagccagaaccccccagtgctgaagaggcaccagagagagatcaccaggactaccctgcagtctgaccaggaggagattgactatgatgacaccatttctgtggagatgaagaaggaggactttgacatttatgatgaggatgagaatcagagccccaggagcttccagaagaagactaggcactattttattgctgctgtggagaggctgtgggactatggcatgagcagctctccccatgtgctgaggaatagggcccagtctggctctgtgcctcagttcaagaaggtggtgttccaggagttcactgatggcagctttacccagcccctgtataggggggagctgaatgagcacctgggcctgctgggcccctatatcagggctgaggtggaggacaatattatggtgacctttaggaaccaggccagcaggccctactctttctatagcagcctgatcagctatgaggaggaccagaggcagggggctgagcccaggaagaattttgtgaagcctaatgagaccaagacctacttctggaaggtgcagcatcacatggcccccaccaaggatgagtttgactgcaaggcttgggcctatttctctgatgtggacctggagaaggatgtgcactctggcctgattggccccctgctggtgtgccacactaacactctgaatcctgcccatggcaggcaggtgactgtgcaggagtttgccctgttcttcaccatctttgatgagaccaagagctggtacttcactgagaacatggagaggaactgcagggccccctgcaacatccagatggaggatcccaccttcaaggagaactacaggtttcatgccatcaatggctacatcatggacactctgcctggcctggtgatggcccaggatcagaggatcaggtggtacctgctgagcatgggctctaatgagaatatccatagcatccacttctctggccatgtgttcactgtcaggaagaaggaggagtacaagatggctctgtataatctgtaccctggggtgtttgagactgtggagatgctgcccagcaaggctggcatctggagggtggagtgcctgattggggagcacctgcatgctgggatgagcaccctgtttctggtgtactctaacaagtgccagacccccctgggcatggcctctgggcacatcagggatttccagatcactgcttctggccagtatggccagtgggcccccaagctggccaggctgcactactctggcagcatcaatgcctggtctaccaaggagcccttttcttggattaaggtggacctgctggcccccatgatcatccatggcatcaagacccagggggccaggcagaagttcagcagcctgtacatcagccagttcatcatcatgtacagcctggatggcaaaaagtggcagacctacaggggcaatagcactgggactctgatggtgttctttggcaatgtggacagctctgggatcaagcacaatatcttcaaccctcccatcattgctaggtacatcaggctgcaccccacccactatagcatcaggtctaccctgaggatggagctgatgggctgtgacctgaactcttgcagcatgcccctgggcatggagtccaaagctatctctgatgcccagattactgccagcagctacttcaccaacatgtttgccacctggtctccctctaaggccaggctgcacctgcagggcaggagcaatgcctggaggccccaggtgaacaatcccaaggagtggctgcaggtggatttccagaaaactatgaaggtgactggggtgaccacccagggggtgaagtctctgctgaccagcatgtatgtgaaggagttcctgatctcttctagccaggatggccaccagtggactctgttcttccagaatggcaaggtgaaggtgttccagggcaaccaggacagcttcacccctgtggtgaactctctggatccccccctgctgaccaggtacctgaggattcatccccagagctgggtgcaccagattgctctgagaatggaggtgctggggtgtgaggctcaggacctgtattga

SEQ ID NO: 12 - DNA, 4374 bp, synthetic construct
  misc_feature 1..4374: note = Description of Artificial Sequence: FVIII Nucleic Acid
  source 1..4374: mol_type = other DNA
atgcagattgagctgtctacttgtttttttctgtgcctgctgaggttctgcttctctgccaccaggaggtattacctgggggctgtggagctgagctgggattacatgcagtctgatctgggggagctgcctgtggatgccaggttcccccccagggtgcccaagagcttccccttcaacacctctgtggtgtataagaagaccctgtttgtggagttcactgatcatctgtttaacattgccaagcccaggcccccctggatgggcctgctgggcccaactatccaggctgaggtgtatgacactgtggtcatcaccctgaagaatatggccagccatcctgtgagcctgcatgctgtgggggtgagctactggaaggcctctgagggggctgagtatgatgaccagaccagccagagggagaaggaggatgacaaggtgttccctgggggcagccacacctatgtgtggcaggtgctgaaggagaatggccccatggcctctgaccccctgtgcctgacttatagctacctgtctcatgtggacctggtgaaggacctgaactctggcctgattggggccctgctggtctgtagggaaggcagcctggccaaggagaagacccagaccctgcacaagtttattctgctgtttgctgtgtttgatgaaggcaagagctggcactctgagaccaagaattctctgatgcaggatagggatgctgcctctgccagggcctggcccaagatgcatactgtgaatggctatgtgaacagaagcctgcctggcctgattggctgccataggaagtctgtgtattggcatgtgattgggatgggcactacccctgaagtgcacagcattttcctggagggccacactttcctggtgaggaaccacaggcaggcctctctggagatcagccccattactttcctgactgcccagaccctgctgatggatctgggccagttcctgctgttctgccacatctctagccaccagcatgatggcatggaggcctatgtgaaggtggacagctgccctgaggagccccagctgaggatgaagaataatgaggaggctgaggattatgatgatgacctgactgactctgagatggatgtggtgaggtttgatgatgataatagccccagcttcatccagatcaggtctgtggccaagaagcatcccaagacctgggtgcactatattgctgctgaagaggaggactgggactatgcccctctggtgctggctcctgatgacaggagctataagagccagtatctgaacaatgggccccagaggattgggaggaagtacaagaaggtgaggttcatggcctacactgatgagacctttaagaccagggaggccatccagcatgagtctggcattctggggcccctgctgtatggggaggtgggggacactctgctgatcattttcaagaaccaggccagcaggccctacaatatttacccccatggcatcactgatgtgaggcccctgtacagcaggaggctgcccaagggggtgaagcacctgaaggacttccccatcctgcctggggagatcttcaagtacaagtggactgtgactgtggaggatggccctaccaagtctgaccctaggtgtctgactaggtactacagcagctttgtgaacatggagagagacctggcttctggcctgattggccccctgctgatctgctacaaggagtctgtggatcagaggggcaaccagattatgtctgataagaggaatgtcatcctgttctctgtgtttgatgagaacaggagctggtatctgactgagaacattcagaggttcctgcccaaccctgctggggtgcagctggaggaccctgagttccaggccagcaacatcatgcattctattaatggctatgtgtttgacagcctgcagctgtctgtgtgcctgcatgaggtggcctactggtacatcctgagcattggggcccagactgactttctgtctgtgtttttctctgggtacaccttcaagcacaagatggtctatgaggacaccctgaccctgttccccttttctggggaaactgtgtttatgagcatggagaaccctgggctgtggatcctgggctgccacaactctgactttaggaataggggcatgactgccctgctgaaggtgagcagctgtgacaagaatactggggattactatgaggacagctatgaggatatctctgcctacctgctgagcaagaacaatgccattgagcctaggagcttcagccagaacccccctgtgctgaagaggcaccagagggagatcaccaggaccaccctgcagtctgatcaggaggagattgactatgatgacaccatctctgtggagatgaagaaggaggactttgatatttatgatgaggatgagaaccagagccccaggagcttccagaagaagaccaggcactatttcattgctgctgtggagaggctgtgggactatggcatgagctctagcccccatgtgctgaggaacagggcccagtctggctctgtgccccagttcaagaaggtggtgttccaggaatttactgatggcagctttacccagcccctgtacagaggggagctgaatgagcacctgggcctgctgggcccctacatcagggctgaggtggaggataatatcatggtgacctttaggaaccaggcctctaggccctattctttttacagcagcctgatcagctatgaggaggaccagaggcagggggctgagcctaggaagaactttgtgaagcccaatgagaccaagacctacttttggaaagtgcagcaccacatggcccccactaaggatgagtttgattgcaaggcctgggcctatttctctgatgtggacctggagaaggatgtgcactctggcctgattggccccctgctggtgtgccacaccaacactctgaaccctgcccatggcaggcaggtgactgtgcaggagtttgccctgttctttaccatctttgatgagactaagagctggtatttcactgagaacatggagaggaactgcagagccccttgcaacatccagatggaggaccctaccttcaaggagaactataggttccatgccatcaatgggtacatcatggataccctgcctggcctggtgatggctcaggaccagaggatcaggtggtacctgctgagcatggggagcaatgagaacattcatagcatccacttctctgggcatgtgttcactgtgaggaagaaggaggagtataagatggccctgtacaacctgtaccctggggtgtttgagactgtggagatgctgcccagcaaggctggcatctggagggtggagtgcctgattggggagcacctgcatgctggcatgagcactctgttcctggtgtacagcaacaagtgccagacccccctgggcatggcctctggccacatcagggacttccagattactgcctctgggcagtatgggcagtgggcccccaagctggccaggctgcactactctgggtctatcaatgcttggagcaccaaggagcctttcagctggatcaaggtggatctgctggcccccatgatcattcatgggatcaagacccagggggccaggcagaagttcagcagcctgtatatttctcagttcatcatcatgtattctctggatggcaaaaagtggcagacctatagagggaacagcactgggaccctgatggtgttttttggcaatgtggatagctctggcatcaagcacaatatcttcaacccccccattattgccaggtacatcaggctgcaccccacccactactctatcaggagcaccctgaggatggagctgatgggctgtgatctgaacagctgctctatgcctctggggatggaaagcaaggccatctctgatgcccagatcactgccagcagctatttcaccaatatgtttgccacttggagccctagcaaggctaggctgcatctgcagggcaggtctaatgcctggaggccccaggtgaacaaccccaaggagtggctgcaggtggacttccagaagactatgaaagtgactggggtgaccacccagggggtgaaaagcctgctgaccagcatgtatgtgaaggagttcctgattagcagcagccaggatggccaccagtggaccctgttcttccagaatgggaaggtgaaggtgtttcagggcaatcaggatagcttcaccccagtggtgaacagcctggacccccccctgctgaccaggtacctgaggatccacccccagagctgggtgcaccagattgccctgaggatggaggtgctgggctgtgaggcccaggatctgtactga

SEQ ID NO: 13 - DNA, 4374 bp, synthetic construct
  misc_feature 1..4374: note = Description of Artificial Sequence: FVIII Nucleic Acid
  source 1..4374: mol_type = other DNA
atgcagattgagctgagcacctgctttttcctgtgcctgctgaggttctgcttctctgctaccaggaggtactacctgggggctgtggagctgtcttgggattacatgcagtctgacctgggggagctgcctgtggatgccaggtttccccccagggtgcccaagtctttcccctttaacacctctgtggtgtataagaagactctgtttgtggagttcactgatcacctgttcaatattgccaagcccaggcccccttggatgggcctgctgggccccactatccaggctgaggtgtatgacactgtggtcatcaccctgaagaacatggccagccaccctgtgagcctgcatgctgtgggggtgagctactggaaggcctctgagggggctgagtatgatgaccagaccagccagagggagaaggaggatgacaaggtgttcccaggggggtctcacacttatgtgtggcaggtgctgaaggagaatgggcccatggcctctgaccctctgtgcctgacttatagctacctgtctcatgtggatctggtgaaggacctgaactctggcctgattggggccctgctggtgtgcagggaggggagcctggccaaggagaagacccagaccctgcacaagttcatcctgctgtttgctgtgtttgatgaggggaagagctggcactctgagaccaagaatagcctgatgcaggacagggatgctgcttctgctagggcctggcctaagatgcacactgtgaatggctatgtgaacaggagcctgcctggcctgattgggtgtcacaggaagtctgtgtactggcatgtgattggcatggggactactccagaagtgcacagcatcttcctggaggggcacaccttcctggtgaggaatcacaggcaggccagcctggagatttctcccatcactttcctgactgcccagaccctgctgatggatctggggcagttcctgctgttctgccacatcagcagccatcagcatgatgggatggaggcctatgtgaaggtggacagctgccctgaggagcctcagctgaggatgaagaacaatgaggaggctgaggactatgatgatgatctgactgactctgagatggatgtggtgaggtttgatgatgacaactctcccagcttcatccagatcaggtctgtggccaagaagcaccccaagacctgggtgcactacattgctgctgaggaggaggattgggattatgctcccctggtgctggctcctgatgataggagctacaagagccagtatctgaataatgggccccagaggattggcaggaagtataagaaggtgaggttcatggcctacactgatgagacctttaagaccagggaggctattcagcatgagtctggcatcctgggccccctgctgtatggggaggtgggggacaccctgctgatcattttcaagaaccaggccagcaggccctataacatctatccccatgggatcactgatgtgaggcccctgtactctaggaggctgcccaagggggtcaagcacctgaaggacttccccatcctgcctggggagatcttcaagtacaagtggactgtgactgtggaggatggccccactaagtctgaccccaggtgcctgactaggtactacagcagctttgtgaacatggagagagatctggcctctggcctgattggccccctgctgatctgctacaaagagtctgtggatcagaggggcaaccagatcatgtctgacaagaggaatgtgatcctgttctctgtgtttgatgagaacagaagctggtacctgactgagaacattcagaggtttctgcccaaccctgctggggtccagctggaggaccctgagtttcaggccagcaacatcatgcacagcatcaatgggtatgtgtttgacagcctgcagctgtctgtgtgcctgcatgaggtggcctactggtatatcctgagcattggggcccagactgatttcctgtctgtgttcttctctggctacactttcaagcacaagatggtgtatgaggataccctgaccctgttccctttctctggggaaactgtgttcatgagcatggagaaccctgggctgtggatcctggggtgccacaattctgatttcaggaacagaggcatgactgctctgctgaaggtgtctagctgtgacaagaacactggggactactatgaggacagctatgaggacatctctgcctacctgctgagcaagaacaatgctattgaacccaggtctttcagccagaacccccctgtgctgaagaggcaccagagggagatcactaggaccaccctgcagtctgatcaggaggagattgactatgatgacaccatctctgtggagatgaagaaggaggactttgacatctatgatgaggatgagaatcagtctcccaggagcttccagaagaagactaggcattacttcattgctgctgtggagaggctgtgggactatggcatgagctctagccctcatgtgctgaggaacagggcccagtctggctctgtgccccagttcaagaaggtggtgtttcaggagttcactgatggcagcttcacccagcccctgtacaggggggagctgaatgagcatctgggcctgctgggcccctacatcagggctgaggtggaggacaacatcatggtgaccttcagaaatcaggctagcaggccctacagcttctacagcagcctgatctcttatgaggaggaccagaggcagggggctgagcccaggaagaactttgtgaagcccaatgagaccaagacctatttctggaaggtgcagcaccacatggcccccaccaaggatgagtttgattgcaaggcctgggcctacttctctgatgtggacctggagaaggatgtgcattctgggctgattggccctctgctggtgtgccacaccaacaccctgaatcctgcccatggcaggcaggtgactgtgcaggagtttgccctgttctttactatctttgatgagaccaagtcttggtattttactgagaacatggagaggaactgcagggccccctgcaacatccagatggaggaccccaccttcaaggagaactacagattccatgccatcaatggctacattatggacactctgcctggcctggtgatggcccaggaccagaggatcaggtggtacctgctgtctatgggcagcaatgagaacattcactctatccacttctctgggcatgtgttcactgtgaggaagaaggaggagtacaagatggccctgtacaacctgtaccctggggtgtttgagactgtggagatgctgcctagcaaggctgggatctggagggtggagtgcctgattggggagcacctgcatgctggcatgtctaccctgttcctggtgtacagcaacaagtgccagacccccctgggcatggcctctggccacatcagagattttcagatcactgcctctggccagtatggccagtgggctcctaagctggccaggctgcactactctggcagcatcaatgcctggagcaccaaggagccctttagctggatcaaggtggacctgctggcccccatgatcatccatggcatcaagactcagggggccaggcagaagttctctagcctgtacattagccagttcatcatcatgtatagcctggatggcaagaagtggcagacctacaggggcaacagcactgggaccctgatggtgttctttgggaatgtggacagctctgggatcaagcacaatatcttcaacccccccattattgccaggtatattaggctgcaccccactcactacagcattaggagcaccctgaggatggagctgatgggctgtgatctgaacagctgcagcatgcccctgggcatggagtctaaggccatctctgatgcccagatcactgccagctcttacttcaccaacatgtttgccacttggagccccagcaaggccaggctgcacctgcagggcaggagcaatgcctggaggccccaggtgaacaaccccaaggagtggctgcaggtggatttccagaagactatgaaggtgactggggtgaccactcagggggtgaagagcctgctgactagcatgtatgtgaaggagttcctgatcagctctagccaggatggccaccagtggaccctgttctttcagaatggcaaggtgaaggtgttccagggcaaccaggactctttcacccctgtggtgaattctctggaccctcccctgctgactaggtatctgaggattcatccccagagctgggtgcatcagattgccctgaggatggaggtgctgggctgtgaggcccaggacctgtattga

SEQ ID NO: 14 - DNA, 4374 bp, synthetic construct
  misc_feature 1..4374: note = Description of Artificial Sequence: FVIII Nucleic Acid
  source 1..4374: mol_type = other DNA
atgcagattgagctgagcacctgcttcttcctgtgcctgctgaggttttgcttttctgccactaggaggtactacctgggggctgtggagctgtcttgggattacatgcagtctgacctgggggagctgccagtggatgccaggttccccccaagggtgcccaagtcttttcccttcaatacctctgtggtgtacaagaagaccctgtttgtggagtttactgatcatctgtttaacattgccaagcccaggcccccctggatggggctgctgggccccaccatccaggctgaggtgtatgatactgtggtgattaccctgaagaatatggccagccatcctgtgtctctgcatgctgtgggggtgtcttattggaaggcctctgagggggctgagtatgatgatcagaccagccagagggagaaggaggatgataaggtgttccctgggggctctcacacctatgtgtggcaggtgctgaaggagaatgggcctatggcctctgacccactgtgcctgacttacagctatctgagccatgtggacctggtgaaggacctgaactctgggctgattggggccctgctggtgtgcagggagggcagcctggccaaggagaagactcagaccctgcacaagttcatcctgctgtttgctgtgtttgatgagggcaagtcttggcactctgagaccaagaacagcctgatgcaggatagggatgctgcctctgccagggcctggcccaagatgcacactgtgaatggctatgtgaacaggtctctgcctggcctgattggctgccacaggaagtctgtgtactggcatgtgattggcatgggcaccacccctgaggtgcatagcattttcctggagggccacaccttcctggtgaggaaccacaggcaggctagcctggagatcagccccatcactttcctgactgcccagaccctgctgatggacctgggccagttcctgctgttctgccacatctctagccaccagcatgatggcatggaggcctatgtgaaggtggactcttgtcctgaggagccccagctgaggatgaagaacaatgaggaggctgaggattatgatgatgatctgactgattctgagatggatgtggtgaggtttgatgatgacaacagcccctctttcatccagatcaggtctgtggccaagaagcaccccaagacctgggtgcactacattgctgctgaggaggaggattgggattatgcccccctggtgctggcccctgatgacaggagctataagtctcagtacctgaacaatggcccccagagaattggcaggaagtacaagaaggtgaggttcatggcctatactgatgagaccttcaaaaccagggaggccattcagcatgagtctggcatcctggggcccctgctgtatggggaggtgggggacaccctgctgatcatcttcaagaaccaggctagcaggccttacaacatctacccccatgggatcactgatgtgaggcccctgtacagcaggaggctgcctaagggggtgaagcacctgaaggactttcccattctgcctggggagatcttcaagtataagtggactgtgactgtggaggatgggcccaccaagtctgaccccaggtgcctgactaggtactactctagctttgtgaacatggagagggacctggcctctgggctgattggccccctgctgatctgttacaaggagtctgtggaccagaggggcaaccagatcatgtctgataagaggaatgtgatcctgttctctgtgtttgatgagaacaggagctggtacctgactgagaacatccagagattcctgcccaaccctgctggggtgcagctggaggatcctgagttccaggccagcaacatcatgcattctatcaatgggtatgtgtttgatagcctgcagctgtctgtgtgtctgcatgaggtggcctactggtacattctgagcattggggcccagactgacttcctgtctgtgttcttctctggctacactttcaaacacaagatggtgtatgaggacaccctgaccctgttccccttctctggggagactgtgtttatgagcatggagaaccctgggctgtggattctgggctgccacaactctgacttcagaaacaggggcatgactgccctgctgaaggtgtcttcttgtgataagaacactggggactattatgaagacagctatgaggacatctctgcctacctgctgagcaagaataatgctattgagcccaggtctttctctcagaacccccctgtgctgaagaggcaccagagggagatcaccaggaccaccctgcagtctgatcaggaggagattgactatgatgacactatttctgtggagatgaagaaggaagactttgatatctatgatgaggatgagaaccagagccctaggagcttccagaagaagactaggcattacttcattgctgctgtggagaggctgtgggactatggcatgagcagcagcccccatgtgctgaggaatagggctcagtctggctctgtgcctcagttcaagaaggtggtgttccaggaattcactgatggcagcttcactcagcccctgtacaggggggagctgaatgagcacctggggctgctgggcccttacatcagggctgaggtggaggacaatatcatggtgacctttaggaaccaggcctctaggccttacagcttctactctagcctgatctcttatgaagaggaccagaggcagggggctgagcccaggaagaactttgtgaagcccaatgagactaagacttacttctggaaggtgcagcaccacatggctcccaccaaggatgagtttgactgcaaggcttgggcctacttctctgatgtggacctggagaaggatgtgcactctgggctgattgggcccctgctggtgtgccacactaacactctgaatcctgcccatggcagacaggtgactgtgcaggagtttgccctgttttttaccatctttgatgagactaagtcttggtacttcactgagaacatggagaggaactgcagggccccctgcaacatccagatggaggatcccaccttcaaggagaactacaggtttcatgccatcaatggctacatcatggacaccctgcctggcctggtgatggctcaggaccagaggattaggtggtatctgctgagcatgggcagcaatgagaatatccactctatccacttctctgggcatgtgttcactgtgaggaagaaggaggagtacaagatggccctgtataacctgtatcctggggtgtttgagactgtggagatgctgcccagcaaggctggcatctggagagtggagtgcctgattggggagcacctgcatgctggcatgagcactctgtttctggtgtatagcaacaagtgtcagacccctctgggcatggcctctgggcacattagggactttcagatcactgcttctggccagtatgggcagtgggctcccaagctggccaggctgcactattctggcagcattaatgcctggagcaccaaggagcctttcagctggatcaaggtggacctgctggcccccatgatcatccatgggatcaagacccagggggctaggcagaagttcagcagcctgtacatcagccagtttatcatcatgtattctctggatggcaagaagtggcagacctacaggggcaattctactggcactctgatggtgttctttgggaatgtggatagctctgggatcaagcataatatcttcaatccccccattattgctaggtatatcaggctgcaccccacccactatagcatcaggagcaccctgaggatggagctgatggggtgtgacctgaacagctgcagcatgcccctgggcatggagagcaaggctatttctgatgcccagatcactgccagcagctactttactaatatgtttgccacctggagccccagcaaggccagactgcacctgcagggcaggtctaatgcctggaggcctcaggtgaataaccccaaggagtggctgcaggtggacttccagaaaaccatgaaggtgactggggtgactacccagggggtgaagtctctgctgaccagcatgtatgtgaaggagttcctgatctcttctagccaggatggccaccagtggaccctgttctttcagaatgggaaggtgaaggtcttccagggcaaccaggatagcttcacccctgtggtgaatagcctggatcctcctctgctgaccaggtatctgaggatccacccccagagctgggtgcatcagattgccctgaggatggaggtgctgggctgtgaggctcaggacctgtactga

SEQ ID NO: 15 - DNA, 4374 bp, synthetic construct
  misc_feature 1..4374: note = Description of Artificial Sequence: FVIII Nucleic Acid
  source 1..4374: mol_type = other DNA
atgcagattgagctgagcacctgtttcttcctgtgcctgctgaggttctgtttctctgccactaggaggtactacctgggggctgtggagctgagctgggactatatgcagtctgacctgggggagctgcctgtggatgccaggttcccccccagggtgcctaagagcttccccttcaatacttctgtggtgtacaagaagactctgtttgtggagtttactgaccacctgttcaacattgctaagcccaggcctccctggatggggctgctgggccccaccatccaggctgaggtgtatgatactgtggtgattaccctgaagaacatggcctctcatccagtgagcctgcatgctgtgggggtgagctactggaaggcctctgaaggggctgagtatgatgaccagaccagccagagggagaaggaggatgacaaggtgttccctgggggcagccacacctatgtgtggcaggtgctgaaggagaatggcccaatggcctctgaccccctgtgcctgacttatagctacctgagccatgtggatctggtgaaggacctgaattctggcctgattggggccctgctggtgtgcagagagggctctctggctaaggagaagacccagactctgcacaagttcatcctgctgtttgctgtgtttgatgagggcaagagctggcactctgagactaagaatagcctgatgcaggacagggatgctgcttctgccagggcctggcccaagatgcatactgtgaatggctatgtgaacaggagcctgcctggcctgattggctgtcacaggaaatctgtctactggcatgtgattgggatgggcactacccctgaggtgcactctatcttcctggagggccataccttcctggtgaggaaccacaggcaggccagcctggagatctctcccattaccttcctgactgcccagaccctgctgatggatctgggccagttcctgctgttctgccacatcagcagccaccagcatgatgggatggaggcttatgtgaaggtggatagctgccctgaggagccccagctgaggatgaagaacaatgaggaggctgaggactatgatgatgacctgactgactctgagatggatgtggtgaggtttgatgatgacaactctcccagctttattcagatcaggtctgtggctaagaagcaccccaagacttgggtgcactacattgctgctgaggaggaggactgggactatgcccctctggtgctggctcctgatgacaggtcttacaagtctcagtacctgaataatggccctcagaggattggcaggaagtacaagaaggtgaggttcatggcctacactgatgagaccttcaagaccagggaggccatccagcatgagtctggcatcctgggccccctgctgtatggggaggtgggggataccctgctgatcatcttcaagaatcaggccagcaggccctacaacatctacccccatggcatcactgatgtgaggccactgtacagcaggaggctgcccaagggggtgaagcatctgaaggacttccccattctgcctggggagatcttcaagtacaaatggactgtgactgtggaggatggccctaccaagtctgaccccaggtgtctgaccaggtactacagcagctttgtgaatatggagagggacctggcctctggcctgattggccccctgctgatctgctacaaggagtctgtggaccagaggggcaatcagatcatgtctgataagaggaatgtgattctgttctctgtgtttgatgagaacaggagctggtacctgactgagaacatccagaggttcctgcccaatcctgctggggtgcagctggaggaccctgagttccaggccagcaatatcatgcacagcatcaatggctatgtctttgacagcctgcagctgtctgtgtgcctgcatgaggtggcttactggtatattctgagcattggggcccagactgatttcctgtctgtgttcttttctggctatacctttaagcacaagatggtgtatgaggacaccctgaccctgttccccttctctggggagactgtgttcatgtctatggagaaccctgggctgtggatcctgggctgccacaactctgacttcaggaacagggggatgactgccctgctgaaggtgtctagctgtgataagaacactggggactattatgaggacagctatgaggacatctctgcttacctgctgagcaagaacaatgccattgagcccaggtctttcagccagaatccccctgtgctgaagaggcatcagagggagatcaccaggaccaccctgcagtctgatcaggaggagattgattatgatgacactatctctgtggaaatgaagaaggaggactttgacatctatgatgaggatgagaaccagagccccaggagcttccagaagaagaccaggcactacttcattgctgctgtggagaggctgtgggattatggcatgagcagctctccccatgtgctgaggaacagagcccagtctggctctgtgcctcagttcaagaaggtggtcttccaggagttcactgatggctctttcacccagcccctgtacaggggggagctgaatgagcacctgggcctgctggggccctacattagggctgaggtggaggataacatcatggtgactttcagaaaccaggccagcaggccttacagcttttactcttctctgattagctatgaggaggatcagaggcagggggctgagcctaggaagaactttgtgaagcccaatgagaccaagacctatttctggaaggtgcagcaccacatggctcccactaaggatgagtttgactgcaaggcttgggcctacttctctgatgtggacctggagaaggatgtgcactctggcctgattgggcccctgctggtgtgccacaccaacaccctgaaccctgcccatggcaggcaggtgactgtgcaggagtttgccctgttcttcaccatctttgatgagactaagagctggtacttcactgagaacatggagaggaactgcagggccccctgcaacatccagatggaggaccccaccttcaaggagaattacaggttccatgccatcaatggctacattatggacaccctgcctggcctggtgatggcccaggatcagaggatcaggtggtatctgctgagcatgggctctaatgagaacatccacagcatccacttctctggccatgtgtttactgtgaggaagaaggaggaatacaagatggctctgtataacctgtaccctggggtgtttgagactgtggagatgctgcccagcaaggctgggatctggagggtggagtgcctgattggggagcacctgcatgctgggatgagcaccctgttcctggtgtatagcaataagtgccagacccccctgggcatggcttctggccacatcagggatttccagatcactgcttctggccagtatggccagtgggctcccaagctggctaggctgcattactctgggtctatcaatgcctggagcactaaggagcccttcagctggatcaaggtggacctgctggcccccatgatcattcatggcatcaagacccagggggctaggcagaagttcagcagcctgtacatcagccagttcatcattatgtacagcctggatggcaagaagtggcagacttacaggggcaatagcactgggactctgatggtgttctttggcaatgtggactcttctggcatcaagcacaacatcttcaaccctcccatcattgccaggtacattaggctgcaccctacccactactctatcaggagcaccctgaggatggagctgatggggtgtgatctgaactcttgcagcatgcctctgggcatggaaagcaaagccatctctgatgcccagatcactgcctctagctatttcaccaatatgtttgccacctggagccctagcaaggccaggctgcacctgcagggcagatctaatgcctggaggccccaggtgaacaatcccaaggagtggctgcaggtggacttccagaagaccatgaaggtgactggggtgaccactcagggggtgaagagcctgctgactagcatgtatgtgaaggagttcctgatctcttctagccaggatggccaccagtggaccctgttcttccagaatggcaaggtgaaagtgttccagggcaaccaggatagcttcactcctgtggtgaactctctggaccctcccctgctgactaggtacctgaggattcatccccagagctgggtgcaccagattgccctgaggatggaggtgctgggctgtgaggcccaggatctgtactga

SEQ ID NO: 16 - DNA, 4374 bp, synthetic construct
  misc_feature 1..4374: note = Description of Artificial Sequence: FVIII Nucleic Acid
  source 1..4374: mol_type = other DNA
atgcagattgagctgagcacctgcttcttcctgtgcctgctgaggttctgcttctctgccaccaggaggtactacctgggggctgtggagctgtcttgggactatatgcagtctgacctgggggagctgccagtggatgccaggttcccccccagggtgcccaagagctttcctttcaacacttctgtggtgtacaagaagaccctgtttgtggagttcactgaccacctgttcaatattgctaagcccaggccaccctggatgggcctgctgggccctaccattcaggctgaggtgtatgacactgtggtgattactctgaagaatatggccagccaccctgtgagcctgcatgctgtgggggtgtcttactggaaggcctctgagggggctgagtatgatgatcagacttctcagagggagaaggaggatgataaggtgttccctgggggctctcacacttatgtgtggcaggtgctgaaggagaatggccccatggcttctgatccactgtgcctgacctactcttacctgagccatgtggacctggtgaaggacctgaactctggcctgattggggccctgctggtgtgcagggagggcagcctggccaaggagaagacccagaccctgcataagttcatcctgctgtttgctgtgtttgatgaggggaagagctggcactctgagaccaagaattctctgatgcaggacagggatgctgcctctgccagggcctggcctaagatgcacactgtgaatggctatgtgaacaggtctctgcctggcctgattggctgccacaggaagtctgtgtactggcatgtgattggcatgggcactacccctgaggtgcacagcattttcctggagggccacaccttcctggtcaggaaccataggcaggcctctctggagatcagccccatcactttcctgactgcccagaccctgctgatggacctgggccagttcctgctgttctgccacattagcagccaccagcatgatggcatggaggcctatgtgaaggtggactcttgccctgaggagccccagctgaggatgaagaacaatgaggaagctgaggattatgatgatgacctgactgactctgagatggatgtggtgaggtttgatgatgacaacagccccagcttcatccagatcaggtctgtggccaagaagcaccccaagacctgggtgcactacattgctgctgaggaggaggattgggactatgctcccctggtgctggctcctgatgataggagctacaagtctcagtacctgaataatggcccccagaggattggcaggaagtacaagaaggtgaggttcatggcctacactgatgagaccttcaagaccagagaggctatccagcatgagtctgggatcctggggcccctgctgtatggggaggtgggggacaccctgctgatcatcttcaagaaccaggccagcagaccctacaacatctacccccatgggatcactgatgtgaggcccctgtacagcaggaggctgcctaagggggtgaagcacctgaaggacttccccatcctgcctggggagatcttcaagtataagtggactgtgactgtggaggatgggcccaccaagtctgaccctaggtgcctgactaggtactactctagctttgtgaacatggagagggacctggcctctggcctgattggccccctgctgatttgctacaaggagtctgtggatcagaggggcaatcagatcatgtctgacaagaggaatgtgatcctgttctctgtgtttgatgagaataggtcttggtacctgactgagaacatccagaggttcctgcctaatcctgctggggtgcagctggaggaccctgagtttcaggccagcaacatcatgcacagcatcaatggctatgtgtttgactctctgcagctgtctgtgtgcctgcatgaggtggcttactggtatatcctgagcattggggctcagactgacttcctgtctgtgttcttttctggctacacttttaagcacaagatggtgtatgaggacaccctgaccctgttccccttttctggggagactgtgttcatgtctatggagaaccctgggctgtggattctgggctgtcacaactctgacttcagaaacaggggcatgactgccctgctgaaggtgtctagctgtgacaagaatactggggactactatgaggacagctatgaggacatttctgcctatctgctgagcaagaacaatgccattgagcccaggagcttttctcagaatccccctgtgctgaagaggcaccagagagagatcaccaggaccactctgcagtctgatcaggaggagattgattatgatgacactatctctgtggagatgaagaaagaggactttgatatctatgatgaggatgagaatcagtctcccaggagcttccagaagaagactagacactacttcattgctgctgtggagaggctgtgggactatggcatgagctctagccctcatgtgctgaggaacagggcccagtctgggtctgtgccccagttcaagaaggtggtgttccaggagttcactgatggcagctttacccagcccctgtataggggggagctgaatgagcatctgggcctgctgggcccctatattagggctgaagtggaggacaacatcatggtgacctttaggaaccaggccagcaggccctacagcttttacagcagcctgattagctatgaggaggatcagagacagggggctgagcccaggaagaactttgtgaagcccaatgagaccaagacctacttctggaaggtgcagcaccacatggcccctaccaaggatgagtttgactgcaaggcctgggcttacttctctgatgtggacctggagaaagatgtgcactctggcctgattgggcccctgctggtgtgccacaccaacaccctgaaccctgcccatgggaggcaggtgactgtgcaggagtttgccctgtttttcaccatctttgatgagaccaagagctggtacttcactgagaacatggagaggaactgcagggccccctgtaacatccagatggaggatcctactttcaaggagaactacaggttccatgccattaatgggtacatcatggacaccctgcctgggctggtgatggcccaggatcagaggattaggtggtatctgctgtctatgggctctaatgagaacatccactctatccacttctctggccatgtgttcactgtgaggaagaaggaggagtacaagatggccctgtacaacctgtaccctggggtgtttgaaactgtggagatgctgccctctaaagctgggatctggagggtggagtgcctgattggggagcacctgcatgctggcatgagcaccctgttcctggtgtacagcaataagtgccagactcccctgggcatggcttctgggcacatcagggatttccagatcactgcctctggccagtatggccagtgggcccccaagctggctaggctgcactactctggcagcatcaatgcctggagcaccaaggagcccttctcttggattaaggtggacctgctggctcccatgatcattcatggcatcaagacccagggggccaggcagaagttttctagcctgtatattagccagttcatcatcatgtatagcctggatgggaagaagtggcagacctacagggggaatagcactggcaccctgatggtgttttttggcaatgtggattcttctggcatcaagcataacatcttcaatccccctatcattgccaggtacattaggctgcatcccacccattactctatcaggagcaccctgaggatggagctgatggggtgtgatctgaacagctgtagcatgcccctgggcatggagtccaaggctatctctgatgcccagatcactgccagcagctacttcaccaacatgtttgccacctggagccccagcaaggccaggctgcacctgcagggcaggtctaatgcctggaggccccaggtgaacaatcccaaggagtggctgcaggtggacttccagaagactatgaaggtgactggggtgaccactcagggggtgaagagcctgctgaccagcatgtatgtgaaggagttcctgatctcttctagccaggatgggcatcagtggaccctgttttttcagaatggcaaagtgaaggtgtttcaggggaatcaggacagctttacccctgtggtgaacagcctggatcctcctctgctgactagatacctgaggatccacccccagagctgggtccaccagattgctctgaggatggaggtgctggggtgtgaggctcaggacctgtactga

SEQ ID NO: 17 - DNA, 4374 bp, synthetic construct
  misc_feature 1..4374: note = Description of Artificial Sequence: FVIII Nucleic Acid
  source 1..4374: mol_type = other DNA
atgcagattgagctgagcacctgcttctttctgtgcctgctgaggttctgcttctctgccaccaggaggtactacctgggggctgtggaactgagctgggactatatgcagtctgacctgggggagctgcctgtggatgccaggttcccccccagggtgcccaagtctttcccctttaacacttctgtggtgtacaagaagaccctgtttgtggagtttactgaccacctgttcaatattgccaagcccaggcccccctggatgggcctgctgggcccaaccatccaggctgaggtgtatgatactgtggtgatcaccctgaagaacatggccagccaccctgtgagcctgcatgctgtgggggtgagctattggaaggcttctgagggggctgagtatgatgaccagactagccagagggagaaggaggatgacaaggtgttccctggggggtctcatacctatgtgtggcaggtgctgaaggagaatggccccatggcctctgaccccctgtgcctgacctattcttacctgagccatgtggacctggtcaaggacctgaactctggcctgattggggctctgctggtgtgcagggagggcagcctggccaaggagaagactcagactctgcataagttcatcctgctgtttgctgtgtttgatgagggcaagagctggcactctgagaccaagaactctctgatgcaggatagggatgctgcctctgccagggcctggcccaagatgcacactgtgaatggctatgtgaataggtctctgcctggcctgattggctgccataggaagtctgtgtactggcatgtgattggcatgggcactacccctgaggtgcactctatcttcctggaggggcacaccttcctggtgaggaaccacaggcaggccagcctggagatctctcccatcaccttcctgactgcccagactctgctgatggacctgggccagttcctgctgttctgccatatcagcagccaccagcatgatggcatggaggcctatgtgaaggtggacagctgcccagaggaaccccagctgaggatgaagaacaatgaggaggctgaggactatgatgatgacctgactgactctgagatggatgtggtgaggtttgatgatgacaacagccccagctttattcagatcaggtctgtggccaagaagcaccccaagacctgggtgcactacattgctgctgaggaggaggactgggattatgcccccctggtgctggcccctgatgacaggtcttacaagtctcagtacctgaacaatggcccccagaggattgggaggaagtacaagaaggtgaggttcatggcctacactgatgagaccttcaagaccagggaggccatccagcatgagtctggcatcctggggcccctgctgtatggggaggtgggggataccctgctgattatcttcaagaaccaggctagcaggccctataacatctacccccatggcattactgatgtgaggcccctgtactctaggagactgcccaagggggtgaagcacctgaaagacttccccatcctgcctggggagatcttcaagtataagtggactgtgactgtggaggatggccccactaagtctgaccccaggtgcctgaccaggtattacagcagctttgtgaatatggagagggatctggcttctggcctgattgggcctctgctgatttgctacaaggagtctgtggatcagagggggaaccagattatgtctgacaagaggaatgtgattctgttctctgtgtttgatgagaacaggagctggtacctgactgagaatatccagaggttcctgcctaatcctgctggggtgcagctggaggaccctgagttccaggctagcaacattatgcacagcatcaatggctatgtgtttgacagcctgcagctgtctgtgtgcctgcatgaggtggcttactggtacattctgtctattggggcccagactgacttcctgtctgtgttcttctctggctacaccttcaagcacaagatggtgtatgaggacactctgaccctgttccccttctctggggagactgtgttcatgagcatggagaatcctgggctgtggattctggggtgccacaactctgatttcaggaacaggggcatgactgccctgctgaaggtgagcagctgtgacaagaacactggggattattatgaggacagctatgaggacatttctgcctacctgctgagcaagaacaatgccattgagcctaggagcttcagccagaatccccctgtgctgaagagacaccagagggagatcactaggaccactctgcagtctgatcaggaggagattgactatgatgacaccatttctgtggagatgaagaaggaggactttgatatttatgatgaggatgagaaccagagccccagaagcttccagaagaagaccaggcactacttcattgctgctgtggagaggctgtgggattatggcatgtcttctagcccccatgtgctgaggaacagggctcagtctggctctgtgcctcagttcaagaaggtggtgttccaggagttcactgatgggagcttcacccagcctctgtacaggggggagctgaatgaacatctgggcctgctggggccctacatcagggctgaggtggaggataatatcatggtgactttcaggaatcaggcctctaggccctacagcttctactctagcctgatcagctatgaggaggaccagaggcagggggctgagcctaggaagaattttgtgaaacccaatgagaccaagacctacttttggaaggtgcagcaccacatggcccctaccaaggatgagtttgactgtaaggcctgggcctacttctctgatgtggacctggagaaggatgtgcattctgggctgattggccccctgctggtgtgccacaccaacaccctgaaccctgcccatggcaggcaggtgactgtgcaggagtttgccctgttcttcaccatctttgatgagactaagagctggtatttcactgagaacatggagaggaactgtagggctccctgcaacatccagatggaggatccaactttcaaggagaactacaggttccatgccatcaatggctacatcatggacaccctgcctggcctggtgatggcccaggaccagaggattaggtggtacctgctgagcatgggctctaatgagaacatccactctatccacttctctggccatgtgtttactgtgaggaagaaggaggagtacaagatggctctgtacaacctgtaccctggggtgtttgagactgtggagatgctgcctagcaaggctggcatttggagagtggagtgtctgattggggagcacctgcatgctgggatgtctaccctgttcctggtgtactctaacaagtgccagacccccctggggatggcttctgggcacatcagagattttcagattactgcttctgggcagtatggccagtgggctcccaagctggccagactgcattactctggctctattaatgcttggagcaccaaggagcctttcagctggatcaaggtggacctgctggctcccatgatcatccatggcattaagactcagggggctaggcagaagttcagcagcctgtatatttctcagtttattatcatgtattctctggatggcaagaagtggcagacttacaggggcaacagcactggcaccctgatggtgttctttggcaatgtggacagctctgggatcaagcataacatcttcaacccccccattattgccaggtacatcaggctgcaccccacccactattctatcaggagcactctgaggatggagctgatggggtgtgacctgaacagctgctctatgcccctgggcatggagagcaaggccatctctgatgcccagatcactgccagctcttatttcaccaacatgtttgccacctggagccccagcaaggccaggctgcacctgcagggcagaagcaatgcctggaggccccaggtgaacaatcctaaggagtggctgcaggtggacttccagaagactatgaaggtgactggggtgactacccagggggtgaagagcctgctgaccagcatgtatgtgaaggagttcctgattagcagcagccaggatgggcatcagtggaccctgttcttccagaatgggaaggtgaaggtgttccagggcaatcaggacagcttcacccctgtggtgaacagcctggacccccccctgctgaccaggtacctgaggatccatccccagagctgggtgcaccagattgctctgagaatggaggtgctgggctgtgaggcccaggacctgtattga

SEQ ID NO: 18 - DNA, 4374 bp, synthetic construct
  misc_feature 1..4374: note = Description of Artificial Sequence: FVIII Nucleic Acid
  source 1..4374: mol_type = other DNA
atgcagattgagctgtctacctgtttttttctgtgcctgctgaggttctgcttctctgctaccaggaggtattatctgggggctgtggagctgagctgggactacatgcagtctgacctgggggagctgcctgtggatgccaggtttcctcccagggtgcctaagagcttccccttcaacacctctgtggtgtacaagaagactctgtttgtggagttcactgaccacctgttcaacattgccaagcccaggcccccctggatggggctgctgggccccactatccaggctgaggtgtatgatactgtggtgattaccctgaagaacatggcctctcaccctgtgtctctgcatgctgtgggggtgagctactggaaggcttctgagggggctgaatatgatgatcagacctctcagagggagaaggaggatgacaaggtgtttcctgggggcagccacacctatgtgtggcaggtgctgaaggagaatgggcccatggcctctgatcccctgtgcctgacctacagctacctgagccatgtggacctggtgaaggacctgaactctggcctgattggggccctgctggtgtgcagggagggcagcctggccaaggaaaagacccagaccctgcataagttcatcctgctgtttgctgtgtttgatgagggcaagtcttggcactctgagaccaagaacagcctgatgcaggacagggatgctgcctctgctagggcctggcccaagatgcacactgtgaatgggtatgtgaacagatctctgcctggcctgattggctgccacaggaagtctgtgtactggcatgtgattggcatggggaccacccctgaggtgcatagcatcttcctggaggggcacaccttcctggtgagaaatcataggcaggccagcctggagattagccccatcaccttcctgactgcccagaccctgctgatggacctgggccagttcctgctgttctgccacatttctagccaccagcatgatggcatggaggcctatgtgaaggtggatagctgccctgaagagccccagctgaggatgaagaacaatgaggaggctgaggattatgatgatgatctgactgactctgagatggatgtggtgaggtttgatgatgacaacagccccagcttcatccagatcaggtctgtggccaagaagcaccctaagacctgggtgcactacattgctgctgaagaggaggactgggactatgcccccctggtgctggccccagatgacaggtcttacaagagccagtacctgaataatggcccccagaggattgggaggaagtataagaaagtgaggttcatggcttacactgatgagacctttaagactagggaggccattcagcatgagtctgggattctgggccctctgctgtatggggaggtgggggacaccctgctgatcattttcaagaaccaggccagcaggccctataatatttatccccatgggattactgatgtcaggcccctgtacagcaggaggctgcctaagggggtgaagcacctgaaggacttccccattctgcctggggagatcttcaagtataagtggactgtgactgtggaggatggccccaccaagtctgatcctaggtgcctgaccaggtactatagcagctttgtgaacatggagagggacctggcttctggcctgattggccccctgctgatctgctacaaggaatctgtggaccagaggggcaaccagattatgtctgacaagaggaatgtgatcctgttttctgtgtttgatgagaataggagctggtatctgactgagaacatccagaggttcctgcccaatcctgctggggtgcagctggaggaccctgagttccaggcttctaacatcatgcatagcatcaatgggtatgtgtttgactctctgcagctgtctgtgtgcctgcatgaggtggcctattggtacatcctgagcattggggcccagactgacttcctgtctgtgttcttctctggctacaccttcaagcacaagatggtgtatgaggacaccctgaccctgttccctttctctggggagactgtgttcatgagcatggagaaccctggcctgtggattctgggctgccataattctgacttcagaaacaggggcatgactgctctgctgaaggtgagcagctgtgacaagaatactggggactactatgaggactcttatgaggatatttctgcctacctgctgagcaagaacaatgctattgagcccaggagcttcagccagaacccccctgtcctgaagaggcatcagagggagatcactaggaccaccctgcagtctgatcaggaggagattgactatgatgacactatctctgtggaaatgaagaaggaggactttgatatctatgatgaggatgagaaccagagccccaggtctttccagaagaagaccaggcactacttcattgctgctgtggagaggctgtgggactatggcatgtctagcagcccccatgtgctgaggaacagagcccagtctggctctgtgccccagttcaagaaggtggtgtttcaggagttcactgatgggagcttcactcagcccctgtataggggggagctgaatgagcatctgggcctgctggggccctacatcagggctgaggtggaggataacatcatggtgaccttcaggaaccaggccagcaggccctactctttctactcttctctgatcagctatgaggaggatcagaggcagggggctgagcctaggaagaactttgtcaagcctaatgagactaagacctacttttggaaggtgcagcaccacatggctcccactaaggatgagtttgattgcaaggcctgggcctacttctctgatgtggacctggagaaggatgtgcactctggcctgattggccccctgctggtgtgtcacaccaataccctgaaccctgcccatggcaggcaggtcactgtgcaggagtttgccctgtttttcactatctttgatgagactaagtcttggtacttcactgagaacatggaaaggaattgcagggctccctgcaacatccagatggaggaccccaccttcaaggagaactacaggtttcatgccatcaatggctacatcatggacaccctgcctggcctggtgatggctcaggatcagaggattaggtggtatctgctgagcatgggcagcaatgagaacatccacagcatccacttttctggccatgtgttcactgtgaggaagaaggaggagtacaagatggctctgtacaatctgtaccctggggtgtttgagactgtggagatgctgcccagcaaggctgggatctggagggtggagtgcctgattggggaacacctgcatgctggcatgtctaccctgttcctggtgtactctaacaagtgccagactcccctgggcatggcctctgggcacatcagggacttccagatcactgcctctgggcagtatggccagtgggcccctaagctggctaggctgcattactctggcagcatcaatgcctggagcaccaaggagcccttcagctggatcaaggtggacctgctggcccctatgatcatccatggcatcaagacccagggggccagacagaagttctcttctctgtacatctctcagttcatcatcatgtactctctggatggcaagaagtggcagacctacagggggaattctactggcactctgatggtgttctttgggaatgtggatagctctgggatcaagcataatattttcaacccccccattattgctaggtacatcaggctgcacccaacccactactctattaggtctaccctgaggatggagctgatgggctgtgacctgaactcttgtagcatgcccctgggcatggagagcaaggctatctctgatgcccagatcactgccagcagctactttaccaacatgtttgctacttggagccccagcaaggccaggctgcacctgcagggcaggagcaatgcctggaggccccaggtgaacaaccccaaggagtggctgcaggtggattttcagaagaccatgaaggtgactggggtgaccactcagggggtgaaaagcctgctgactagcatgtatgtgaaggagtttctgatcagcagctctcaggatggccatcagtggaccctgttcttccagaatggcaaggtgaaggtgttccagggcaaccaggatagcttcacccctgtggtgaatagcctggacccccccctgctgaccaggtacctgaggatccatccccagagctgggtgcaccagattgccctgaggatggaggtgctgggctgtgaagcccaggacctgtactga

SEQ ID NO: 19 - DNA, 4374 bp, synthetic construct
  misc_feature 1..4374: note = Description of Artificial Sequence: FVIII Nucleic Acid
  source 1..4374: mol_type = other DNA
atgcaaatagagctctccacctgcttctttctgtgccttttgcgattctgctttagtgccaccagaagatactacctgggtgcagtggaactgtcatgggactatatgcaaagtgatctcggtgagctgcctgtggacgcaagatttcctcctagagtgccaaaatcttttccattcaacacctcagtcgtgtacaaaaagactctgtttgtagaattcacggatcaccttttcaacatcgctaagccaaggccaccctggatgggtctgctaggtcctaccatccaggctgaggtttatgatacagtggtcattacacttaagaacatggcttcccatcctgtcagtcttcatgctgttggtgtatcctactggaaagcttctgagggagctgaatatgatgatcagaccagtcaaagggagaaagaagatgataaagtcttccctggtggaagccatacatatgtctggcaggtcctgaaagagaatggtccaatggcctctgacccactgtgccttacctactcatatctttctcatgtggacctggtaaaagacttgaattcaggcctcattggagccctactagtatgtagagaagggagtctggccaaggaaaagacacagaccttgcacaaatttatactactttttgctgtatttgatgaagggaaaagttggcactcagaaacaaagaactccttgatgcaggatagggatgctgcatctgctcgggcctggcctaaaatgcacacagtcaatggttatgtaaacaggtctctgccaggtctgattggatgccacaggaaatcagtctattggcatgtgattggaatgggcaccactcctgaagtgcactcaatattcctcgaaggtcacacatttcttgtgaggaaccatcgccaggcgtccttggaaatctcgccaataactttccttactgctcaaacactcttgatggaccttggacagtttctactgttttgtcatatctcttcccaccaacatgatggcatggaagcttatgtcaaagtagacagctgtccagaggaaccccaactacgaatgaaaaataatgaagaagcggaagactatgatgatgatcttactgattctgaaatggatgtggtcaggtttgatgatgacaactctccttcctttatccaaattcgctcagttgccaagaagcatcctaaaacttgggtacattacattgctgctgaagaggaggactgggactatgctcccttagtcctcgcccccgatgacagaagttataaaagtcaatatttgaacaatggccctcagcggattggtaggaagtacaaaaaagtccgatttatggcatacacagatgaaacctttaagactcgtgaagctattcagcatgaatcaggaatcttgggacctttactttatggggaagttggagacacactgttgattatatttaagaatcaagcaagcagaccatataacatctaccctcacggaatcactgatgtccgtcctttgtattcaaggagattaccaaaaggtgtaaaacatttgaaggattttccaattctgccaggagaaatattcaaatataaatggacagtgactgtagaagatgggccaactaaatcagatcctcggtgcctgacccgctattactctagtttcgttaatatggagagagatctagcttcaggactcattggccctctcctcatctgctacaaagaatctgtagatcaaagaggaaaccagataatgtcagacaagaggaatgtcatcctgttttctgtatttgatgagaaccgaagctggtacctcacagagaatatacaacgctttctccccaatccagctggagtgcagcttgaggatccagagttccaagcctccaacatcatgcacagcatcaatggctatgtttttgatagtttgcagttgtcagtttgtttgcatgaggtggcatactggtacattctaagcattggagcacagactgacttcctttctgtcttcttctctggatataccttcaaacacaaaatggtctatgaagacacactcaccctattcccattctcaggagaaactgtcttcatgtcgatggaaaacccaggtctatggattctggggtgccacaactcagactttcggaacagaggcatgaccgccttactgaaggtttctagttgtgacaagaacactggtgattattacgaggacagttatgaagatatttcagcatacttgctgagtaaaaacaatgccattgaaccaagaagcttctcccaaaacccaccagtcttgaaacgccatcaacgggaaataactcgtactactcttcagtcagatcaagaggaaattgactatgatgataccatatcagttgaaatgaagaaggaagattttgacatttatgatgaggatgaaaatcagagcccccgcagctttcaaaagaaaacacgacactattttattgctgcagtggagaggctctgggattatgggatgagtagctccccacatgttctaagaaacagggctcagagtggcagtgtccctcagttcaagaaagttgttttccaggaatttactgatggctcctttactcagcccttataccgtggagaactaaatgaacatttgggactcctggggccatatataagagcagaagttgaagataatatcatggtaactttcagaaatcaggcctctcgtccctattccttctattctagccttatttcttatgaggaagatcagaggcaaggagcagaacctagaaaaaactttgtcaagcctaatgaaaccaaaacttacttttggaaagtgcaacatcatatggcacccactaaagatgagtttgactgcaaagcctgggcttatttctctgatgttgacctggaaaaagatgtgcactcaggcctgattggaccccttctggtctgccacactaacacactgaaccctgctcatgggagacaagtgacagtacaggaatttgctctgtttttcaccatctttgatgagaccaaaagctggtacttcactgaaaatatggaaagaaactgcagggctccctgcaatatccagatggaagatcccacttttaaagagaattatcgcttccatgcaatcaatggctacataatggatacactacctggcttagtaatggctcaggatcaaaggattcgatggtatctgctcagcatgggcagcaatgaaaacatccattctattcatttcagtggacatgtgttcaccgtacgaaaaaaagaggagtataaaatggcactgtacaatctctatccaggtgtttttgagacagtggaaatgttaccatccaaagctggaatttggcgggtggaatgccttattggcgagcatctacatgctgggatgagcacactttttctggtgtacagcaataagtgtcagactcccctgggaatggcttctggacacattagagattttcagattacagcttcaggacaatatggacagtgggccccaaagctggccagacttcattattccggatcaatcaatgcctggagcaccaaggagcccttttcttggatcaaggtggatctgttggcaccaatgattattcacggcatcaagacccagggtgcccgtcagaagttctccagcctctacatctctcagtttatcatcatgtatagtcttgatgggaagaagtggcagacttatcgaggaaattccactggaaccttaatggtcttctttggcaatgtggattcatctgggataaaacacaatatttttaaccctccaattattgctcgatacatccgtttgcacccaactcattatagcattcgcagcactcttcgcatggagttgatgggctgtgatttaaatagttgcagcatgccattgggaatggagagtaaagcaatatcagatgcacagattactgcttcatcctactttaccaatatgtttgccacctggtctccttcaaaagctcgacttcacctccaagggaggagtaatgcctggagacctcaggtgaataatccaaaagagtggctgcaagtggacttccagaagacaatgaaagtcacaggagtaactactcagggagtaaaatctctgcttaccagcatgtatgtgaaggagttcctcatctccagcagtcaagatggccatcagtggactctcttttttcagaatggcaaagtaaaggtttttcagggaaatcaagactccttcacacctgtggtgaactctctagacccaccgttactgactcgctaccttcgaattcacccccagagttgggtgcaccagattgccctgaggatggaggttctgggctgcgaggcacaggacctctactga

SEQ ID NO: 20 - DNA, 4890 bp, synthetic construct
  misc_feature 1..4890: note = Description of Artificial Sequence: FVIII Nucleic Acid
  source 1..4890: mol_type = other DNA
atgcagattgagctgagcacctgcttcttcctgtgcctgctgaggttctgcttctctgccaccaggagatactacctgggggctgtggagctgagctgggactacatgcagtctgacctgggggagctgcctgtggatgccaggttcccccccagagtgcccaagagcttccccttcaacacctctgtggtgtacaagaagaccctgtttgtggagttcactgaccacctgttcaacattgccaagcccaggcccccctggatgggcctgctgggccccaccatccaggctgaggtgtatgacactgtggtgatcaccctgaagaacatggccagccaccctgtgagcctgcatgctgtgggggtgagctactggaaggcctctgagggggctgagtatgatgaccagaccagccagagggagaaggaggatgacaaggtgttccctgggggcagccacacctatgtgtggcaggtgctgaaggagaatggccccatggcctctgaccccctgtgcctgacctacagctacctgagccatgtggacctggtgaaggacctgaactctggcctgattggggccctgctggtgtgcagggagggcagcctggccaaggagaagacccagaccctgcacaagttcatcctgctgtttgctgtgtttgatgagggcaagagctggcactctgaaaccaagaacagcctgatgcaggacagggatgctgcctctgccagggcctggcccaagatgcacactgtgaatggctatgtgaacaggagcctgcctggcctgattggctgccacaggaagtctgtgtactggcatgtgattggcatgggcaccacccctgaggtgcacagcatcttcctggagggccacaccttcctggtcaggaaccacaggcaggccagcctggagatcagccccatcaccttcctgactgcccagaccctgctgatggacctgggccagttcctgctgttctgccacatcagcagccaccagcatgatggcatggaggcctatgtgaaggtggacagctgccctgaggagccccagctgaggatgaagaacaatgaggaggctgaggactatgatgatgacctgactgactctgagatggatgtggtgaggtttgatgatgacaacagccccagcttcatccagatcaggtctgtggccaagaagcaccccaagacctgggtgcactacattgctgctgaggaggaggactgggactatgcccccctggtgctggcccctgatgacaggagctacaagagccagtacctgaacaatggcccccagaggattggcaggaagtacaagaaggtcaggttcatggcctacactgatgaaaccttcaagaccagggaggccatccagcatgagtctggcatcctgggccccctgctgtatggggaggtgggggacaccctgctgatcatcttcaagaaccaggccagcaggccctacaacatctacccccatggcatcactgatgtgaggcccctgtacagcaggaggctgcccaagggggtgaagcacctgaaggacttccccatcctgcctggggagatcttcaagtacaagtggactgtgactgtggaggatggccccaccaagtctgaccccaggtgcctgaccagatactacagcagctttgtgaacatggagagggacctggcctctggcctgattggccccctgctgatctgctacaaggagtctgtggaccagaggggcaaccagatcatgtctgacaagaggaatgtgatcctgttctctgtgtttgatgagaacaggagctggtacctgactgagaacatccagaggttcctgcccaaccctgctggggtgcagctggaggaccctgagttccaggccagcaacatcatgcacagcatcaatggctatgtgtttgacagcctgcagctgtctgtgtgcctgcatgaggtggcctactggtacatcctgagcattggggcccagactgacttcctgtctgtgttcttctctggctacaccttcaagcacaagatggtgtatgaggacaccctgaccctgttccccttctctggggagactgtgttcatgagcatggagaaccctggcctgtggattctgggctgccacaactctgacttcaggaacaggggcatgactgccctgctgaaagtctccagctgtgacaagaacactggggactactatgaggacagctatgaggacatctctgcctacctgctgagcaagaacaatgccattgagcccaggagcttcagccagaacagcaggcaccccagcaccaggcagaagcagttcaatgccaccaccatccctgagaatgacatagagaagacagacccatggtttgcccaccggacccccatgcccaagatccagaatgtgagcagctctgacctgctgatgctgctgaggcagagccccaccccccatggcctgagcctgtctgacctgcaggaggccaagtatgaaaccttctctgatgaccccagccctggggccattgacagcaacaacagcctgtctgagatgacccacttcaggccccagctgcaccactctggggacatggtgttcacccctgagtctggcctgcagctgaggctgaatgagaagctgggcaccactgctgccactgagctgaagaagctggacttcaaagtctccagcaccagcaacaacctgatcagcaccatcccctctgacaacctggctgctggcactgacaacaccagcagcctgggcccccccagcatgcctgtgcactatgacagccagctggacaccaccctgtttggcaagaagagcagccccctgactgagtctgggggccccctgagcctgtctgaggagaacaatgacagcaagctgctggagtctggcctgatgaacagccaggagagcagctggggcaagaatgtgagcaccaggagcttccagaagaagaccaggcactacttcattgctgctgtggagaggctgtgggactatggcatgagcagcagcccccatgtgctgaggaacagggcccagtctggctctgtgccccagttcaagaaggtggtgttccaggagttcactgatggcagcttcacccagcccctgtacagaggggagctgaatgagcacctgggcctgctgggcccctacatcagggctgaggtggaggacaacatcatggtgaccttcaggaaccaggccagcaggccctacagcttctacagcagcctgatcagctatgaggaggaccagaggcagggggctgagcccaggaagaactttgtgaagcccaatgaaaccaagacctacttctggaaggtgcagcaccacatggcccccaccaaggatgagtttgactgcaaggcctgggcctacttctctgatgtggacctggagaaggatgtgcactctggcctgattggccccctgctggtgtgccacaccaacaccctgaaccctgcccatggcaggcaggtgactgtgcaggagtttgccctgttcttcaccatctttgatgaaaccaagagctggtacttcactgagaacatggagaggaactgcagggccccctgcaacatccagatggaggaccccaccttcaaggagaactacaggttccatgccatcaatggctacatcatggacaccctgcctggcctggtgatggcccaggaccagaggatcaggtggtacctgctgagcatgggcagcaatgagaacatccacagcatccacttctctggccatgtgttcactgtgaggaagaaggaggagtacaagatggccctgtacaacctgtaccctggggtgtttgagactgtggagatgctgcccagcaaggctggcatctggagggtggagtgcctgattggggagcacctgcatgctggcatgagcaccctgttcctggtgtacagcaacaagtgccagacccccctgggcatggcctctggccacatcagggacttccagatcactgcctctggccagtatggccagtgggcccccaagctggccaggctgcactactctggcagcatcaatgcctggagcaccaaggagcccttcagctggatcaaggtggacctgctggcccccatgatcatccatggcatcaagacccagggggccaggcagaagttcagcagcctgtacatcagccagttcatcatcatgtacagcctggatggcaagaagtggcagacctacaggggcaacagcactggcaccctgatggtgttctttggcaatgtggacagctctggcatcaagcacaacatcttcaacccccccatcattgccagatacatcaggctgcaccccacccactacagcatcaggagcaccctgaggatggagctgatgggctgtgacctgaacagctgcagcatgcccctgggcatggagagcaaggccatctctgatgcccagatcactgccagcagctacttcaccaacatgtttgccacctggagccccagcaaggccaggctgcacctgcagggcaggagcaatgcctggaggccccaggtcaacaaccccaaggagtggctgcaggtggacttccagaagaccatgaaggtgactggggtgaccacccagggggtgaagagcctgctgaccagcatgtatgtgaaggagttcctgatcagcagcagccaggatggccaccagtggaccctgttcttccagaatggcaaggtgaaggtgttccagggcaaccaggacagcttcacccctgtggtgaacagcctggacccccccctgctgaccagatacctgaggattcacccccagagctgggtgcaccagattgccctgaggatggaggtgctgggctgtgaggcccaggacctgtactga

SEQ ID NO: 21 - DNA, 4374 bp, synthetic construct
  misc_feature 1..4374: note = Description of Artificial Sequence: FVIII Nucleic Acid
  source 1..4374: mol_type = other DNA
atgcagattgagctgtcaacttgctttttcctgtgcctgctgagattttgtttttccgctactagaagatactacctgggggctgtggaactgtcttgggattacatgcagagtgacctgggagagctgccagtggacgcacgatttccacctagagtccctaaatcattccccttcaacaccagcgtggtctataagaaaacactgttcgtggagtttactgatcacctgttcaacatcgctaagcctcggccaccctggatgggactgctgggaccaacaatccaggcagaggtgtacgacaccgtggtcattacactgaaaaacatggcctcacaccccgtgagcctgcatgctgtgggcgtcagctactggaaggcttccgaaggggcagagtatgacgatcagacttcccagagagaaaaagaggacgataaggtgtttcctggcgggtctcatacctatgtgtggcaggtcctgaaagagaatggccccatggcttccgaccctctgtgcctgacctactcttatctgagtcacgtggacctggtcaaggatctgaacagcggactgatcggagcactgctggtgtgtagggaagggagcctggctaaggagaaaacccagacactgcataagttcattctgctgttcgccgtgtttgacgaaggaaaatcatggcacagcgagacaaagaatagtctgatgcaggaccgggatgccgcttcagccagagcttggcccaaaatgcacactgtgaacggctacgtcaatcgctcactgcctggactgatcggctgccaccgaaagagcgtgtattggcatgtcatcggaatgggcaccacacctgaagtgcactccattttcctggaggggcatacctttctggtccgcaaccaccgacaggcctccctggagatctctccaattaccttcctgacagctcagactctgctgatggatctgggacagttcctgctgttttgccacatcagctcccaccagcatgatggcatggaggcctacgtgaaagtggacagctgtcccgaggaacctcagctgaggatgaagaacaatgaggaagctgaagactatgacgatgacctgaccgactccgagatggatgtggtccgattcgatgacgataacagcccctcctttatccagattagatctgtggccaagaaacaccctaagacatgggtccattacatcgcagccgaggaagaggactgggattatgcaccactggtgctggcaccagacgatcgatcctacaaatctcagtatctgaacaatggaccacagcggattggcagaaagtacaagaaagtgaggttcatggcttataccgatgaaaccttcaagactcgcgaagcaatccagcacgagagcgggattctgggaccactgctgtacggagaagtgggggacaccctgctgatcatttttaagaaccaggccagcaggccttacaatatctatccacatggaattacagatgtgcgccctctgtacagccggagactgccaaagggcgtcaaacacctgaaggacttcccaatcctgcccggggaaatttttaagtataaatggactgtcaccgtcgaggatggccccactaagagcgaccctaggtgcctgacccgctactattctagtttcgtgaatatggaaagggatctggccagcggactgatcggcccactgctgatttgttacaaagagagcgtggatcagagaggcaaccagatcatgtccgacaagaggaatgtgattctgttcagtgtctttgacgaaaaccggtcatggtatctgaccgagaacatccagagattcctgcctaatccagccggagtgcagctggaagatcctgagtttcaggcttctaacatcatgcatagtattaatggctacgtgttcgacagtctgcagctgtcagtgtgtctgcacgaggtcgcttactggtatatcctgagcattggagcacagacagatttcctgagcgtgttcttttccggctacacttttaagcataaaatggtgtatgaggacacactgactctgttccccttcagcggcgaaaccgtgtttatgtccatggagaatcccgggctgtggatcctgggatgccacaacagcgatttcaggaatcgcgggatgactgccctgctgaaagtgtcaagctgtgacaagaacaccggagactactatgaagattcatacgaggacatcagcgcatatctgctgtccaaaaacaatgccattgaacccaggtcttttagtcagaatcctccagtgctgaagaggcaccagcgcgagatcacccgcactaccctgcagagtgatcaggaagagatcgactacgacgatacaatttctgtggaaatgaagaaagaggacttcgatatctatgacgaagatgagaaccagagtcctcgatcattccagaagaaaacccggcattactttattgctgcagtggagcgcctgtgggattatggcatgtcctctagtcctcacgtgctgcgaaatcgggcccagtcagggagcgtcccacagttcaagaaagtggtcttccaggagtttacagacggatcctttactcagccactgtaccggggcgaactgaacgagcacctggggctgctgggaccctatatcagagctgaagtggaggataacattatggtcaccttcagaaatcaggcatctaggccttacagtttttattcaagcctgatctcttacgaagaggaccagaggcagggagcagaaccacgaaaaaacttcgtgaagcctaatgagaccaaaacatacttttggaaggtgcagcaccatatggccccaacaaaagacgaattcgattgcaaggcatgggcctatttttctgacgtggatctggagaaggacgtccacagtggcctgatcgggccactgctggtgtgtcatactaacaccctgaatcccgcacacggcaggcaggtcactgtccaggaattcgccctgttctttaccatctttgatgagacaaaaagctggtacttcaccgaaaacatggagcgaaattgccgggctccatgtaatattcagatggaagaccccacattcaaggagaactaccgctttcatgccatcaatgggtatattatggatactctgcccggactggtcatggctcaggaccagagaatcaggtggtacctgctgagcatggggtccaacgagaatatccactcaattcatttcagcggacacgtgtttactgtccggaagaaagaagagtataaaatggccctgtacaacctgtatcccggcgtgttcgaaaccgtcgagatgctgcctagcaaggcagggatctggagagtggaatgcctgattggggagcacctgcatgccggaatgtctaccctgtttctggtgtacagtaataagtgtcagacacccctggggatggcttccggacatatccgggatttccagattaccgcatctggacagtacggccagtgggcccctaagctggctagactgcactattccgggtctatcaacgcttggtccacaaaagagcctttctcttggattaaggtggacctgctggcaccaatgatcattcatggcatcaaaactcagggggccaggcagaagttctcctctctgtacatctcacagtttatcatcatgtacagcctggatggcaagaaatggcagacataccgcggcaatagcacagggactctgatggtgttctttggcaacgtggacagttcagggatcaagcacaacattttcaatccccctatcattgctagatacatcaggctgcacccaacccattattctattcgaagtacactgcggatggaactgatggggtgcgatctgaacagttgttcaatgcccctgggaatggagtccaaggcaatctctgacgcccagattaccgctagctcctacttcactaatatgtttgctacctggagcccctccaaagcacgactgcatctgcagggacgaagcaacgcatggcgaccacaggtgaacaatcccaaggagtggctgcaggtcgattttcagaaaactatgaaggtgaccggagtcacaactcagggcgtgaaaagtctgctgacctcaatgtacgtcaaggagttcctgatctctagttcacaggacggccaccagtggacactgttctttcagaacggaaaggtgaaagtcttccagggcaatcaggattcctttacacctgtggtcaactctctggacccacccctgctgactcgctacctgcgaatccacccacagtcctgggtgcatcagattgcactgagaatggaagtcctgggctgcgaggcccaggacctgtattga

SEQ ID NO: 22 - DNA, 222 bp, synthetic construct
  misc_feature 1..222: note = Description of Artificial Sequence: TTR Promoter
  source 1..222: mol_type = other DNA
gtctgtctgcacatttcgtagagcgagtgttccgatactctaatctccctaggcaaggttcatattgacttaggttacttattctccttttgttgactaagtcaataatcagaatcagcaggtttggagtcagcttggcagggatcagcagcctgggttggaaggagggggtataaaagccccttcaccaggagaagccgtcacacagatccacaagctcct

SEQ ID NO: 23 - DNA, 5066 bp, synthetic construct
  misc_feature 1..5066: note = Description of Artificial Sequence: Expression Cassette
  source 1..5066: mol_type = other DNA
cctgcaggcagctgcgcgctcgctcgctcactgaggccgcccgggcaaagcccgggcgtcgggcgacctttggtcgcccggcctcagtgagcgagcgagcgcgcagagagggagtggccaactccatcactaggggttcctacgcgtgtctgtctgcacatttcgtagagcgagtgttccgatactctaatctccctaggcaaggttcatattgacttaggttacttattctccttttgttgactaagtcaataatcagaatcagcaggtttggagtcagcttggcagggatcagcagcctgggttggaaggagggggtataaaagccccttcaccaggagaagccgtcacacagatccacaagctcctgctagcaggtaagtgccgtgtgtggttcccgcgggcctggcctctttacgggttatggcccttgcgtgccttgaattactgacactgacatccactttttctttttctccacaggtttaaacgccaccatgcagattgagctgagcacctgcttcttcctgtgtctgctgaggttctgcttctctgccaccaggaggtattacctgggggctgtggagctgagctgggactatatgcagtctgacctgggggagctgcctgtggatgctaggttcccccccagggtgcccaagagcttcccctttaacacttctgtggtgtacaagaagaccctgtttgtggagttcactgaccacctgttcaacattgccaagcccaggcccccctggatggggctgctggggcccaccatccaggctgaggtgtatgacactgtggtgatcaccctgaagaacatggccagccaccctgtgagcctgcatgctgtgggggtgagctactggaaggcttctgagggggctgagtatgatgaccagactagccagagggagaaggaggatgacaaggtgtttcctgggggcagccatacctatgtgtggcaggtgctgaaggagaatggccccatggcctctgaccccctgtgcctgacctacagctacctgtctcatgtggacctggtgaaggacctgaactctggcctgattggggctctgctggtgtgtagggagggcagcctggctaaggaaaagacccagaccctgcataagtttatcctgctgtttgctgtgtttgatgagggcaagagctggcactctgagaccaagaacagcctgatgcaggatagggatgctgcctctgccagggcttggcctaagatgcacactgtgaatgggtatgtgaataggagcctgcctggcctgattggctgccacaggaagtctgtgtactggcatgtgattgggatgggcaccacccctgaggtccatagcatcttcctggagggccacactttcctggtgaggaaccacagacaggcctctctggagatctctcccatcaccttcctgactgctcagactctgctgatggacctgggccagttcctgctgttttgccatattagcagccaccagcatgatgggatggaggcctatgtgaaggtggatagctgccctgaggagcctcagctgaggatgaagaacaatgaggaggctgaagactatgatgatgacctgactgattctgagatggatgtggtgaggtttgatgatgacaatagccccagcttcattcagatcaggtctgtggccaagaaacaccccaagacctgggtgcactacattgctgctgaggaagaggactgggactatgctcccctggtgctggcccctgatgataggtcttataagagccagtacctgaacaatgggccccagaggattggcaggaagtacaagaaggtgaggttcatggcctacactgatgaaaccttcaaaaccagggaggccattcagcatgagtctggcatcctgggccctctgctgtatggggaggtgggggacaccctgctgatcatcttcaagaaccaggccagcaggccctacaacatctatcctcatggcatcactgatgtgaggcccctgtacagcaggaggctgcccaagggggtgaagcacctgaaagacttccccatcctgcctggggagatctttaagtataagtggactgtgactgtggaggatggccctaccaagtctgaccccaggtgtctgaccaggtactattctagctttgtgaacatggagagggacctggcctctggcctgattgggcccctgctgatctgctacaaggagtctgtggaccagaggggcaaccagatcatgtctgacaagaggaatgtgatcctgttttctgtgtttgatgagaataggagctggtacctgactgagaacatccagaggtttctgcccaatcctgctggggtgcagctggaggatcctgagttccaggccagcaatatcatgcatagcatcaatggctatgtgtttgacagcctgcagctgtctgtgtgcctgcatgaggtggcctactggtacatcctgagcattggggcccagactgactttctgtctgtgttcttttctggctataccttcaagcacaagatggtgtatgaggataccctgaccctgttccccttctctggggagactgtgttcatgagcatggagaatcctgggctgtggatcctggggtgccacaactctgattttaggaacagggggatgactgccctgctgaaggtgtctagctgtgataagaacactggggactactatgaggacagctatgaggacatttctgcttatctgctgtctaagaataatgccattgagcccagaagcttcagccagaatccccctgtgctgaagagacatcagagggagatcaccagaactaccctgcagtctgatcaggaggagattgactatgatgacactatctctgtggagatgaagaaggaggactttgacatctatgatgaggatgagaatcagtctcccaggagctttcagaagaagaccagacattacttcattgctgctgtggagaggctgtgggactatggcatgagctctagccctcatgtgctgaggaacagggcccagtctggctctgtgccccagttcaagaaggtggtgttccaggaattcactgatggcagcttcacccagcccctgtacaggggggagctgaatgagcacctgggcctgctggggccttatatcagggctgaggtggaggataatattatggtgactttcaggaaccaggccagcaggccctactctttctatagcagcctgatctcttatgaggaggatcagaggcagggggctgagcctaggaagaactttgtgaagcccaatgagactaagacctacttctggaaggtccagcaccacatggcccctaccaaggatgagtttgactgcaaggcctgggcctatttctctgatgtggatctggagaaggatgtccattctgggctgattggccccctgctggtgtgccacactaacactctgaatcctgcccatggcaggcaggtgactgtccaggagtttgccctgttcttcactatctttgatgagaccaagagctggtactttactgagaacatggagaggaactgcagagctccttgcaatattcagatggaggaccccaccttcaaggagaattacaggttccatgccattaatgggtacatcatggacaccctgcctggcctggtgatggctcaggaccagaggatcaggtggtacctgctgagcatgggctctaatgagaatatccacagcatccacttctctgggcatgtgttcactgtgaggaagaaggaggagtacaagatggctctgtataatctgtaccctggggtgtttgaaactgtggagatgctgccctctaaggctggcatctggagggtggagtgcctgattggggagcacctgcatgctggcatgagcaccctgttcctggtgtacagcaacaagtgccagacccccctgggcatggcctctggccacatcagggacttccagatcactgcctctggccagtatggccagtgggcccccaagctggccaggctgcactattctggcagcatcaatgcctggagcaccaaggagcccttcagctggatcaaggtggacctgctggcccccatgatcattcatggcatcaagacccagggggccaggcagaagttcagctctctgtacatctctcagttcatcatcatgtactctctggatgggaagaagtggcagacctacaggggcaacagcactggcaccctgatggtgttctttgggaatgtggactcttctggcatcaagcacaacatcttcaatccccccatcattgctaggtatattaggctgcatcccacccactacagcatcaggtctaccctgaggatggagctgatgggctgtgacctgaactcttgcagcatgcccctgggcatggagtctaaggccatctctgatgcccagattactgccagcagctacttcaccaacatgtttgccacctggagcccctctaaggccaggctgcatctgcaggggaggagcaatgcctggaggcctcaggtgaacaaccccaaggagtggctgcaggtggatttccagaagaccatgaaggtgactggggtgaccacccagggggtcaagagcctgctgaccagcatgtatgtgaaggagttcctgatcagcagcagccaggatggccaccagtggactctgttctttcagaatgggaaggtgaaggtgtttcagggcaatcaggactctttcacccctgtggtgaacagcctggacccccccctgctgaccagatacctgaggatccacccccagtcttgggtgcatcagattgccctgaggatggaggtgctgggctgtgaggctcaggatctgtactgagcggccgcaataaaagatcagagctctagagatctgtgtgttggttttttgtgtaggaacccctagtgatggagttggccactccctctctgcgcgctcgctcgctcactgaggccgggcgaccaaaggtcgcccgacgcccgggctttgcccgggcggcctcagtgagcgagcgagcgcgcagctgcctgcagg

SEQ ID NO: 24 - DNA, 11976 bp, synthetic construct
  misc_feature 1..11976: note = Description of Artificial Sequence: Plasmid
  source 1..11976: mol_type = other DNA
cctgcaggcagctgcgcgctcgctcgctcactgaggccgcccgggcaaagcccgggcgtcgggcgacctttggtcgcccggcctcagtgagcgagcgagcgcgcagagagggagtggccaactccatcactaggggttcctacgcgtgtctgtctgcacatttcgtagagcgagtgttccgatactctaatctccctaggcaaggttcatattgacttaggttacttattctccttttgttgactaagtcaataatcagaatcagcaggtttggagtcagcttggcagggatcagcagcctgggttggaaggagggggtataaaagccccttcaccaggagaagccgtcacacagatccacaagctcctgctagcaggtaagtgccgtgtgtggttcccgcgggcctggcctctttacgggttatggcccttgcgtgccttgaattactgacactgacatccactttttctttttctccacaggtttaaacgccaccatgcagattgagctgagcacctgcttcttcctgtgtctgctgaggttctgcttctctgccaccaggaggtattacctgggggctgtggagctgagctgggactatatgcagtctgacctgggggagctgcctgtggatgctaggttcccccccagggtgcccaagagcttcccctttaacacttctgtggtgtacaagaagaccctgtttgtggagttcactgaccacctgttcaacattgccaagcccaggcccccctggatggggctgctggggcccaccatccaggctgaggtgtatgacactgtggtgatcaccctgaagaacatggccagccaccctgtgagcctgcatgctgtgggggtgagctactggaaggcttctgagggggctgagtatgatgaccagactagccagagggagaaggaggatgacaaggtgtttcctgggggcagccatacctatgtgtggcaggtgctgaaggagaatggccccatggcctctgaccccctgtgcctgacctacagctacctgtctcatgtggacctggtgaaggacctgaactctggcctgattggggctctgctggtgtgtagggagggcagcctggctaaggaaaagacccagaccctgcataagtttatcctgctgtttgctgtgtttgatgagggcaagagctggcactctgagaccaagaacagcctgatgcaggatagggatgctgcctctgccagggcttggcctaagatgcacactgtgaatgggtatgtgaataggagcctgcctggcctgattggctgccacaggaagtctgtgtactggcatgtgattgggatgggcaccacccctgaggtccatagcatcttcctggagggccacactttcctggtgaggaaccacagacaggcctctctggagatctctcccatcaccttcctgactgctcagactctgctgatggacctgggccagttcctgctgttttgccatattagcagccaccagcatgatgggatggaggcctatgtgaaggtggatagctgccctgaggagcctcagctgaggatgaagaacaatgaggaggctgaagactatgatgatgacctgactgattctgagatggatgtggtgaggtttgatgatgacaatagccccagcttcattcagatcaggtctgtggccaagaaacaccccaagacctgggtgcactacattgctgctgaggaagaggactgggactatgctcccctggtgctggcccctgatgataggtcttataagagccagtacctgaacaatgggccccagaggattggcaggaagtacaagaaggtgaggttcatggcctacactgatgaaaccttcaaaaccagggaggccattcagcatgagtctggcatcctgggccctctgctgtatggggaggtgggggacaccctgctgatcatcttcaagaaccaggccagcaggccctacaacatctatcctcatggcatcactgatgtgaggcccctgtacagcaggaggctgcccaagggggtgaagcacctgaaagacttccccatcctgcctggggagatctttaagtataagtggactgtgactgtggaggatggccctaccaagtctgaccccaggtgtctgaccaggtactattctagctttgtgaacatggagagggacctggcctctggcctgattgggcccctgctgatctgctacaaggagtctgtggaccagaggggcaaccagatcatgtctgacaagaggaatgtgatcctgttttctgtgtttgatgagaataggagctggtacctgactgagaacatccagaggtttctgcccaatcctgctggggtgcagctggaggatcctgagttccaggccagcaatatcatgcatagcatcaatggctatgtgtttgacagcctgcagctgtctgtgtgcctgcatgaggtggcctactggtacatcctgagcattggggcccagactgactttctgtctgtgttcttttctggctataccttcaagcacaagatggtgtatgaggataccctgaccctgttccccttctctggggagactgtgttcatgagcatggagaatcctgggctgtggatcctggggtgccacaactctgattttaggaacagggggatgactgccctgctgaaggtgtctagctgtgataagaacactggggactactatgaggacagctatgaggacatttctgcttatctgctgtctaagaataatgccattgagcccagaagcttcagccagaatccccctgtgctgaagagacatcagagggagatcaccagaactaccctgcagtctgatcaggaggagattgactatgatgacactatctctgtggagatgaagaaggaggactttgacatctatgatgaggatgagaatcagtctcccaggagctttcagaagaagaccagacattacttcattgctgctgtggagaggctgtgggactatggcatgagctctagccctcatgtgctgaggaacagggcccagtctggctctgtgccccagttcaagaaggtggtgttccaggaattcactgatggcagcttcacccagcccctgtacaggggggagctgaatgagcacctgggcctgctggggccttatatcagggctgaggtggaggataatattatggtgactttcaggaaccaggccagcaggccctactctttctatagcagcctgatctcttatgaggaggatcagaggcagggggctgagcctaggaagaactttgtgaagcccaatgagactaagacctacttctggaaggtccagcaccacatggcccctaccaaggatgagtttgactgcaaggcctgggcctatttctctgatgtggatctggagaaggatgtccattctgggctgattggccccctgctggtgtgccacactaacactctgaatcctgcccatggcaggcaggtgactgtccaggagtttgccctgttcttcactatctttgatgagaccaagagctggtactttactgagaacatggagaggaactgcagagctccttgcaatattcagatggaggaccccaccttcaaggagaattacaggttccatgccattaatgggtacatcatggacaccctgcctggcctggtgatggctcaggaccagaggatcaggtggtacctgctgagcatgggctctaatgagaatatccacagcatccacttctctgggcatgtgttcactgtgaggaagaaggaggagtacaagatggctctgtataatctgtaccctggggtgtttgaaactgtggagatgctgccctctaaggctggcatctggagggtggagtgcctgattggggagcacctgcatgctggcatgagcaccctgttcctggtgtacagcaacaagtgccagacccccctgggcatggcctctggccacatcagggacttccagatcactgcctctggccagtatggccagtgggcccccaagctggccaggctgcactattctggcagcatcaatgcctggagcaccaaggagcccttcagctggatcaaggtggacctgctggcccccatgatcattcatggcatcaagacccagggggccaggcagaagttcagctctctgtacatctctcagttcatcatcatgtactctctggatgggaagaagtggcagacctacaggggcaacagcactggcaccctgatggtgttctttgggaatgtggactcttctggcatcaagcacaacatcttcaatccccccatcattgctaggtatattaggctgcatcccacccactacagcatcaggtctaccctgaggatggagctgatgggctgtgacctgaactcttgcagcatgcccctgggcatggagtctaaggccatctctgatgcccagattactgccagcagctacttcaccaacatgtttgccacctggagcccctctaaggccaggctgcatctgcaggggaggagcaatgcctggaggcctcaggtgaacaaccccaaggagtggctgcaggtggatttccagaagaccatgaaggtgactggggtgaccacccagggggtcaagagcctgctgaccagcatgtatgtgaaggagttcctgatcagcagcagccaggatggccaccagtggactctgttctttcagaatgggaaggtgaaggtgtttcagggcaatcaggactctttcacccctgtggtgaacagcctggacccccccctgctgaccagatacctgaggatccacccccagtcttgggtgcatcagattgccctgaggatggaggtgctgggctgtgaggctcaggatctgtactgagcggccgcaataaaagatcagagctctagagatctgtgtgttggttttttgtgtaggaacccctagtgatggagttggccactccctctctgcgcgctcgctcgctcactgaggccgggcgaccaaaggtcgcccgacgcccgggctttgcccgggcggcctcagtgagcgagcgagcgcgcagctgcctgcaggggcagcttgaaggaaatactaaggcaaaggtactgcaagtgctcgcaacattcgcttatgcggattattgccgtagtgccgcgacgccgggggcaagatgcagagattgccatggtacaggccgtgcggttgatattgccaaaacagagctgtgggggagagttgtcgagaaagagtgcggaagatgcaaaggcgtcggctattcaaggatgccagcaagcgcagcatatcgcgctgtgacgatgctaatcccaaaccttacccaacccacctggtcacgcactgttaagccgctgtatgacgctctggtggtgcaatgccacaaagaagagtcaatcgcagacaacattttgaatgcggtcacacgttagcagcatgattgccacggatggcaacatattaacggcatgatattgacttattgaataaaattgggtaaatttgactcaacgatgggttaattcgctcgttgtggtagtgagatgaaaagaggcggcgcttactaccgattccgcctagttggtcacttcgacgtatcgtctggaactccaaccatcgcaggcagagaggtctgcaaaatgcaatcccgaaacagttcgcaggtaatagttagagcctgcataacggtttcgggattttttatatctgcacaacaggtaagagcattgagtcgataatcgtgaagagtcggcgagcctggttagccagtgctctttccgttgtgctgaattaagcgaataccggaagcagaaccggatcaccaaatgcgtacaggcgtcatcgccgcccagcaacagcacaacccaaactgagccgtagccactgtctgtcctgaattcattagtaatagttacgctgcggccttttacacatgaccttcgtgaaagcgggtggcaggaggtcgcgctaacaacctcctgccgttttgcccgtgcatatcggtcacgaacaaatctgattactaaacacagtagcctggatttgttctatcagtaatcgaccttattcctaattaaatagagcaaatccccttattgggggtaagacatgaagatgccagaaaaacatgacctgttggccgccattctcgcggcaaaggaacaaggcatcggggcaatccttgcgtttgcaatggcgtaccttcgcggcagatataatggcggtgcgtttacaaaaacagtaatcgacgcaacgatgtgcgccattatcgcctagttcattcgtgaccttctcgacttcgccggactaagtagcaatctcgcttatataacgagcgtgtttatcggctacatcggtactgactcgattggttcgcttatcaaacgcttcgctgctaaaaaagccggagtagaagatggtagaaatcaataatcaacgtaaggcgttcctcgatatgctggcgtggtcggagggaactgataacggacgtcagaaaaccagaaatcatggttatgacgtcattgtaggcggagagctatttactgattactccgatcaccctcgcaaacttgtcacgctaaacccaaaactcaaatcaacaggcgccggacgctaccagcttctttcccgttggtgggatgcctaccgcaagcagcttggcctgaaagacttctctccgaaaagtcaggacgctgtggcattgcagcagattaaggagcgtggcgctttacctatgattgatcgtggtgatatccgtcaggcaatcgaccgttgcagcaatatctgggcttcactgccgggcgctggttatggtcagttcgagcataaggctgacagcctgattgcaaaattcaaagaagcgggcggaacggtcagagagattgatgtatgagcagagtcaccgcgattatctccgctctggttatctgcatcatcgtctgcctgtcatgggctgttaatcattaccgtgataacgccattacctacaaagcccagcgcgacaaaaatgccagagaactgaagctggcgaacgcggcaattactgacatgcagatgcgtcagcgtgatgttgctgcgctcgatgcaaaatacacgaaggagttagctgatgctaaagctgaaaatgatgctctgcgtgatgatgttgccgctggtcgtcgtcggttgcacatcaaagcagtctgtcagtcagtgcgtgaagccaccaccgcctccggcgtggataatgcagcctccccccgactggcagacaccgctgaacgggattatttcaccctcagagagaggctgatcactatgcaaaaacaactggaaggaacccagaagtatattaatgagcagtgcagatagagttgcccatatcgatgggcaactcatgcaattattgtgagcaatacacacgcgcttccagcggagtataaatgcctaaagtaataaaaccgagcaatccatttacgaatgtttgctgggtttctgttttaacaacattttctgcgccgccacaaattttggctgcatcgacagttttcttctgcccaattccagaaacgaagaaatgatgggtgatggtttcctttggtgctactgctgccggtttgttttgaacagtaaacgtctgttgagcacatcctgtaataagcagggccagcgcagtagcgagtagcatttttttcatggtgttattcccgatgctttttgaagttcgcagaatcgtatgtgtagaaaattaaacaaaccctaaacaatgagttgaaatttcatattgttaatatttattaatgtatgtcaggtgcgatgaatcgtcattgtattcccggattaactatgtccacagccctgacggggaacttctctgcgggagtgtccgggaataattaaaacgatgcacacagggtttagcgcgtacacgtattgcattatgccaacgccccggtgctgacacggaagaaaccggacgttatgatttagcgtggaaagatttgtgtagtgttctgaatgctctcagtaaatagtaatgaattatcaaaggtatagtaatatcttttatgttcatggatatttgtaacccatcggaaaactcctgctttagcaagattttccctgtattgctgaaatgtgatttctcttgatttcaacctatcataggacgtttctataagatgcgtgtttcttgagaatttaacatttacaacctttttaagtccttttattaacacggtgttatcgttttctaacacgatgtgaatattatctgtggctagatagtaaatataatgtgagacgttgtgacgttttagttcagaataaaacaattcacagtctaaatcttttcgcacttgatcgaatatttctttaaaaatggcaacctgagccattggtaaaaccttccatgtgatacgagggcgcgtagtttgcattatcgtttttatcgtttcaatctggtctgacctccttgtgttttgttgatgatttatgtcaaatattaggaatgttttcacttaatagtattggttgcgtaacaaagtgcggtcctgctggcattctggagggaaatacaaccgacagatgtatgtaaggccaacgtgctcaaatcttcatacagaaagatttgaagtaatattttaaccgctagatgaagagcaagcgcatggagcgacaaaatgaataaagaacaatctgctgatgatccctccgtggatctgattcgtgtaaaaaatatgcttaatagcaccatttctatgagttaccctgatgttgtaattgcatgtatagaacataaggtgtctctggaagcattcagagcaattgaggcagcgttggtgaagcacgataataatatgaaggattattccctggtggttgactgatcaccataactgctaatcattcaaactatttagtctgtgacagagccaacacgcagtctgtcactgtcaggaaagtggtaaaactgcaactcaattactgcaatgccctcgtaattaagtgaatttacaatatcgtcctgttcggagggaagaacgcgggatgttcattcttcatcacttttaattgatgtatatgctctcttttctgacgttagtctccgacggcaggcttcaatgacccaggctgagaaattcccggaccctttttgctcaagagcgatgttaatttgttcaatcatttggttaggaaagcggatgttgcgggttgttgttctgcgggttctgttcttcgttgacatgaggttgccccgtattcagtgtcgctgatttgtattgtctgaagttgtttttacgttaagttgatgcagatcaattaatacgatacctgcgtcataattgattatttgacgtggtttgatggcctccacgcacgttgtgatatgtagatgataatcattatcactttacgggtcctttccggtgatccgacaggttacggggcggcgacctgcctgatgcggtattttctccttacgcatctgtgcggtatttcacaccgcatacgtcaaagcaaccatagtacgcgccctgtagcggcgcattaagcgcggcgggtgtggtggttacgcgcagcgtgaccgctacacttgccagcgccttagcgcccgctcctttcgctttcttcccttcctttctcgccacgttcgccggctttccccgtcaagctctaaatcgggggctccctttagggttccgatttagtgctttacggcacctcgaccccaaaaaacttgatttgggtgatggttcacgtagtgggccatcgccctgatagacggtttttcgccctttgacgttggagtccacgttctttaatagtggactcttgttccaaactggaacaacactcaactctatctcgggctattcttttgatttagacctgcaggcatgcaagcttggcactggccgtcgttttacaacgtcgtgactgggaaaaccctggcgttacccaacttaatcgccttgcagcacatccccctttcgccagctggcgtaatagcgaagaggcccgcaccgatcgcccttcccaacagttgcgcagcctgaatggcgaatgcgatttattcaacaaagccgccgtcccgtcaagtcagcgtaatgctctgccagtgttacaaccaattaaccaattctgattagaaaaactcatcgagcatcaaatgaaactgcaatttattcatatcaggattatcaataccatatttttgaaaaagccgtttctgtaatgaaggagaaaactcaccgaggcagttccataggatggcaagatcctggtatcggtctgcgattccgactcgtccaacatcaatacaacctattaatttcccctcgtcaaaaataaggttatcaagtgagaaatcaccatgagtgacgactgaatccggtgagaatggcaaaagcttatgcatttctttccagacttgttcaacaggccagccattacgctcgtcatcaaaatcactcgcatcaaccaaaccgttattcattcgtgattgcgcctgagcgagacgaaatacgcgatcgctgttaaaaggacaattacaaacaggaatcgaatgcaaccggcgcaggaacactgccagcgcatcaacaatattttcacctgaatcaggatattcttctaatacctggaatgctgttttcccggggatcgcagtggtgagtaaccatgcatcatcaggagtacggataaaatgcttgatggtcggaagaggcataaattccgtcagccagtttagtctgaccatctcatctgtaacatcattggcaacgctacctttgccatgtttcagaaacaactctggcgcatcgggcttcccatacaatcgatagattgtcgcacctgattgcccgacattatcgcgagcccatttatacccatataaatcagcatccatgttggaatttaatcgcggcttcgagcaagacgtttcccgttgaatatggctcataacaccccttgtattactgtttatgtaagcagacagttttattgttcatgatgatatatttttatcttgtgcaatgtaacatcagagattttgagacacaacgtggctttgttgaataaatcgaacttttgctgagttgaaggatcagatcacgcatcttcccgacaacgcagaccgttccgtggcaaagcaaaagttcaaaatcaccaactggtccacctacaacaaagctctcatcaaccgtggctccctcactttctggctggatgatggggcgattcaggcctggtatgagtcagcaacaccttcttcacgaggcagacctctcgacggagttccactgagcgtcagaccccgtagaaaagatcaaaggatcttcttgagatcctttttttctgcgcgtaatctgctgcttgcaaacaaaaaaaccaccgctaccagcggtggtttgtttgccggatcaagagctaccaactctttttccgaaggtaactggcttcagcagagcgcagataccaaatactgttcttctagtgtagccgtagttaggccaccacttcaagaactctgtagcaccgcctacatacctcgctctgctaatcctgttaccagtggctgctgccagtggcgataagtcgtgtcttaccgggttggactcaagacgatagttaccggataaggcgcagcggtcgggctgaacggggggttcgtgcacacagcccagcttggagcgaacgacctacaccgaactgagatacctacagcgtgagctatgagaaagcgccacgcttcccgaagggagaaaggcggacaggtatccggtaagcggcagggtcggaacaggagagcgcacgagggagcttccagggggaaacgcctggtatctttatagtcctgtcgggtttcgccacctctgacttgagcgtcgatttttgtgatgctcgtcaggggggcggagcctatggaaaaacgccagcaacgcggcctttttacggttcctggccttttgctggccttttgctcacatgt

SEQ ID NO: 25 - protein, 1457 aa, synthetic construct
  REGION 1..1457: note = Description of Artificial Sequence: FVIII Peptide
MQIELSTCFFLCLLRFCFSATRRYYLGAVELSWDYMQSDLGELPVDARFPPRVPKSFPFNTSVVYKKTLFVEFTDHLFNIAKPRPPWMGLLGPTIQAEVYDTVVITLKNMASHPVSLHAVGVSYWKASEGAEYDDQTSQREKEDDKVFPGGSHTYVWQVLKENGPMASDPLCLTYSYLSHVDLVKDLNSGLIGALLVCREGSLAKEKTQTLHKFILLFAVFDEGKSWHSETKNSLMQDRDAASARAWPKMHTVNGYVNRSLPGLIGCHRKSVYWHVIGMGTTPEVHSIFLEGHTFLVRNHRQASLEISPITFLTAQTLLMDLGQFLLFCHISSHQHDGMEAYVKVDSCPEEPQLRMKNNEEAEDYDDDLTDSEMDVVRFDDDNSPSFIQIRSVAKKHPKTWVHYIAAEEEDWDYAPLVLAPDDRSYKSQYLNNGPQRIGRKYKKVRFMAYTDETFKTREAIQHESGILGPLLYGEVGDTLLIIFKNQASRPYNIYPHGITDVRPLYSRRLPKGVKHLKDFPILPGEIFKYKWTVTVEDGPTKSDPRCLTRYYSSFVNMERDLASGLIGPLLICYKESVDQRGNQIMSDKRNVILFSVFDENRSWYLTENIQRFLPNPAGVQLEDPEFQASNIMHSINGYVFDSLQLSVCLHEVAYWYILSIGAQTDFLSVFFSGYTFKHKMVYEDTLTLFPFSGETVFMSMENPGLWILGCHNSDFRNRGMTALLKVSSCDKNTGDYYEDSYEDISAYLLSKNNAIEPRSFSQNPPVLKRHQREITRTTLQSDQEEIDYDDTISVEMKKEDFDIYDEDENQSPRSFQKKTRHYFIAAVERLWDYGMSSSPHVLRNRAQSGSVPQFKKVVFQEFTDGSFTQPLYRGELNEHLGLLGPYIRAEVEDNIMVTFRNQASRPYSFYSSLISYEEDQRQGAEPRKNFVKPNETKTYFWKVQHHMAPTKDEFDCKAWAYFSDVDLEKDVHSGLIGPLLVCHTNTLNPAHGRQVTVQEFALFFTIFDETKSWYFTENMERNCRAPCNIQMEDPTFKENYRFHAINGYIMDTLPGLVMAQDQRIRWYLLSMGSNENIHSIHFSGHVFTVRKKEEYKMALYNLYPGVFETVEMLPSKAGIWRVECLIGEHLHAGMSTLFLVYSNKCQTPLGMASGHIRDFQITASGQYGQWAPKLARLHYSGSINAWSTKEPFSWIKVDLLAPMIIHGIKTQGARQKFSSLYISQFIIMYSLDGKKWQTYRGNSTGTLMVFFGNVDSSGIKHNIFNPPIIARYIRLHPTHYSIRSTLRMELMGCDLNSCSMPLGMESKAISDAQITASSYFTNMFATWSPSKARLHLQGRSNAWRPQVNNPKEWLQVDFQKTMKVTGVTTQGVKSLLTSMYVKEFLISSSQDGHQWTLFFQNGKVKVFQGNQDSFTPVVNSLDPPLLTRYLRIHPQSWVHQIALRMEVLGCEAQDLY

SEQ ID NO: 26 - protein, 2351 aa, synthetic construct
  REGION 1..2351: note = Description of Artificial Sequence: FVIII Peptide
MQIELSTCFFLCLLRFCFSATRRYYLGAVELSWDYMQSDLGELPVDARFPPRVPKSFPFNTSVVYKKTLFVEFTDHLFNIAKPRPPWMGLLGPTIQAEVYDTVVITLKNMASHPVSLHAVGVSYWKASEGAEYDDQTSQREKEDDKVFPGGSHTYVWQVLKENGPMASDPLCLTYSYLSHVDLVKDLNSGLIGALLVCREGSLAKEKTQTLHKFILLFAVFDEGKSWHSETKNSLMQDRDAASARAWPKMHTVNGYVNRSLPGLIGCHRKSVYWHVIGMGTTPEVHSIFLEGHTFLVRNHRQASLEISPITFLTAQTLLMDLGQFLLFCHISSHQHDGMEAYVKVDSCPEEPQLRMKNNEEAEDYDDDLTDSEMDVVRFDDDNSPSFIQIRSVAKKHPKTWVHYIAAEEEDWDYAPLVLAPDDRSYKSQYLNNGPQRIGRKYKKVRFMAYTDETFKTREAIQHESGILGPLLYGEVGDTLLIIFKNQASRPYNIYPHGITDVRPLYSRRLPKGVKHLKDFPILPGEIFKYKWTVTVEDGPTKSDPRCLTRYYSSFVNMERDLASGLIGPLLICYKESVDQRGNQIMSDKRNVILFSVFDENRSWYLTENIQRFLPNPAGVQLEDPEFQASNIMHSINGYVFDSLQLSVCLHEVAYWYILSIGAQTDFLSVFFSGYTFKHKMVYEDTLTLFPFSGETVFMSMENPGLWILGCHNSDFRNRGMTALLKVSSCDKNTGDYYEDSYEDISAYLLSKNNAIEPRSFSQNSRHPSTRQKQFNATTIPENDIEKTDPWFAHRTPMPKIQNVSSSDLLMLLRQSPTPHGLSLSDLQEAKYETFSDDPSPGAIDSNNSLSEMTHFRPQLHHSGDMVFTPESGLQLRLNEKLGTTAATELKKLDFKVSSTSNNLISTIPSDNLAAGTDNTSSLGPPSMPVHYDSQLDTTLFGKKSSPLTESGGPLSLSEENNDSKLLESGLMNSQESSWGKNVSSTESGRLFKGKRAHGPALLTKDNALFKVSISLLKTNKTSNNSATNRKTHIDGPSLLIENSPSVWQNILESDTEFKKVTPLIHDRMLMDKNATALRLNHMSNKTTSSKNMEMVQQKKEGPIPPDAQNPDMSFFKMLFLPESARWIQRTHGKNSLNSGQGPSPKQLVSLGPEKSVEGQNFLSEKNKVVVGKGEFTKDVGLKEMVFPSSRNLFLTNLDNLHENNTHNQEKKIQEEIEKKETLIQENVVLPQIHTVTGTKNFMKNLFLLSTRQNVEGSYDGAYAPVLQDFRSLNDSTNRTKKHTAHFSKKGEEENLEGLGNQTKQIVEKYACTTRISPNTSQQNFVTQRSKRALKQFRLPLEETELEKRIIVDDTSTQWSKNMKHLTPSTLTQIDYNEKEKGAITQSPLSDCLTRSHSIPQANRSPLPIAKVSSFPSIRPIYLTRVLFQDNSSHLPAASYRKKDSGVQESSHFLQGAKKNNLSLAILTLEMTGDQREVGSLGTSATNSVTYKKVENTVLPKPDLPKTSGKVELLPKVHIYQKDLFPTETSNGSPGHLDLVEGSLLQGTEGAIKWNEANRPGKVPFLRVATESSAKTPSKLLDPLAWDNHYGTQIPKEEWKSQEKSPEKTAFKKKDTILSLNACESNHAIAAINEGQNKPEIEVTWAKQGRTERLCSQNPPVLKRHQREITRTTLQSDQEEIDYDDTISVEMKKEDFDIYDEDENQSPRSFQKKTRHYFIAAVERLWDYGMSSSPHVLRNRAQSGSVPQFKKVVFQEFTDGSFTQPLYRGELNEHLGLLGPYIRAEVEDNIMVTFRNQASRPYSFYSSLISYEEDQRQGAEPRKNFVKPNETKTYFWKVQHHMAPTKDEFDCKAWAYFSDVDLEKDVHSGLIGPLLVCHTNTLNPAHGRQVTVQEFALFFTIFDETKSWYFTENMERNCRAPCNIQMEDPTFKENYRFHAINGYIMDTLPGLVMAQDQRIRWYLLSMGSNENIHSIHFSGHVFTVRKKEEYKMALYNLYPGVFETVEMLPSKAGIWRVECLIGEHLHAGMSTLFLVYSNKCQTPLGMASGHIRDFQITASGQYGQWAPKLARLHYSGSINAWSTKEPFSWIKVDLLAPMIIHGIKTQGARQKFSSLYISQFIIMYSLDGKKWQTYRGNSTGTLMVFFGNVDSSGIKHNIFNPPIIARYIRLHPTHYSIRSTLRMELMGCDLNSCSMPLGMESKAISDAQITASSYFTNMFATWSPSKARLHLQGRSNAWRPQVNNPKEWLQVDFQKTMKVTGVTTQGVKSLLTSMYVKEFLISSSQDGHQWTLFFQNGKVKVFQGNQDSFTPVVNSLDPPLLTRYLRIHPQSWVHQIALRMEVLGCEAQDLY

SEQ ID NO: 27 - protein, 736 aa, synthetic construct
  REGION 1..736: note = Description of Artificial Sequence: AAV Capsid
MAADGYLPDWLEDNLSEGIREWWALQPGAPKPKANQQHQDNARGLVLPGYKYLGPGNGLDKGEPVNAADAAALEHDKAYDQQLKAGDNPYLKYNHADAEFQERLKEDTSFGGNLGRAVFQAKKRLLEPLGLVEEAAKTAPGKKRPVDQSPQEPDSSSGVGKSGKQPARKRLNFGQTGDSESVPDPQPLGEPPAAPTSLGSNTMASGGGAPMADNNEGADGVGNSSGNWHCDSQWLGDRVITTSTRTWALPTYNNHLYKQISSQSGASNDNHYFGYSTPWGYFDFNRFHCHFSPRDWQRLINNNWGFRPKKLSFKLFNIQVKEVTQNDGTTTIANNLTSTVQVFTDSEYQLPYVLGSAHQGCLPPFPADVFMVPQYGYLTLNNGSQAVGRSSFYCLEYFPSQMLRTGNNFQFSYTFEDVPFHSSYAHSQSLDRLMNPLIDQYLYYLNRTQGTTSGTTNQSRLLFSQAGPQSMSLQARNWLPGPCYRQQRLSKTANDNNNSNFPWTAASKYHLNGRDSLVNPGPAMASHKDDEEKFFPMHGNLIFGKEGTTASNAELDNVMITDEEEIRTTNPVATEQYGTVANNLQSSNTAPTTRTVNDQGALPGMVWQDRDVYLQGPIWAKIPHTDGHFHPSPLMGGFGLKHPPPQIMIKNTPVPANPPTTFSPAKFASFITQYSTGQVSVEIEWELQKENSKRWNPEIQYTSNYNKSVNVDFTVDTNGVYSEPRPIGTRYLTRPL

SEQ ID NO: 28 - protein, 738 aa, synthetic construct
  REGION 1..738: note = Description of Artificial Sequence: AAV Capsid
MAADGYLPDWLEDNLSEGIREWWDLKPGAPKPKANQQKQDNGRGLVLPGYKYLGPFNGLDKGEPVNAADAAALEHDKAYDQQLQAGDNPYLRYNHADAEFQERLQEDTSFGGNLGRAVFQAKKRVLEPLGLVESPVKTAPGKKRPVEPSPQRSPDSSTGIGKKGQQPAKKRLNFGQTGDSESVPDPQPIGEPPAAPSGVGPNTMAAGGGAPMADNNEGADGVGSSSGNWHCDSTWLGDRVITTSTRTWALPTYNNHLYKQISNGTSGGSTNDNTYFGYSTPWGYFDFNRFHCHFSPRDWQRLINNNWGFRPKRLNFKLFNIQVKEVTQNEGTKTIANNLTSTIQVFTDSEYQLPYVLGSAHQGCLPPFPADVFMIPQYGYLTLNNGSQAVGRSSFYCLEYFPSQMLRTGNNFEFSYNFEDVPFHSSYAHSQSLDRLMNPLIDQYLYYLSRTQSTGGTAGTQQLLFSQAGPNNMSAQAKNWLPGPCYRQQRVSTTLSQNNNSNFAWTGATKYHLNGRDSLVNPGVAMATHKDDEERFFPSSGVLMFGKQGAGKDNVDYSSVMLTSEEEIKTTNPVATEQYGVVADNLQQQNAAPIVGAVNSQGALPGMVWQNRDVYLQGPIWAKIPHTDGNFHPSPLMGGFGLKHPPPQILIKNTPVPADPPTTFNQAKLASFITQYSTGQVSVEIEWELQKENSKRWNPEIQYTSNYYKSTNVDFAVNTEGTYSEPRPIGTRYLTRNL

SEQ ID NO: 29 - protein, 14 aa, synthetic construct
  REGION 1..14: note = Description of Artificial Sequence: FVIII Peptide
SFSQNPPVLKRHQR